European Patent Specification EP 3 390 425 B1, published August 7, 2024. Title: DIETARY PEPTIDES. Applicant: Diet4Life ApS. The sequence listing filed with the application follows.

SEQUENCE LISTING (1005 sequences)

SEQ ID NO: 1 - protein, 8 aa, Artificial Sequence
  Artificial peptide sequence
  MISC_FEATURE (1)..(1): Xaa in position 1 is A, L, I, or V
  MISC_FEATURE (2)..(2): Xaa in position 2 is S, T, G, A, N, E or D
  MISC_FEATURE (3)..(3): Xaa in position 3 is D, E, or G
  MISC_FEATURE (5)..(5): Xaa in position 5 is P, N, S, D, A, T, K, or G
  MISC_FEATURE (6)..(6): Xaa in position 6 is Y, N, I, W, or F
  MISC_FEATURE (7)..(7): Xaa in position 7 is I, L, R, or V
  MISC_FEATURE (8)..(8): Xaa in position 8 is L, I, V, S, M, or T
XXXKXXXX

SEQ ID NO: 2 - protein, 8 aa, Artificial Sequence
  Artificial peptide sequence
  MISC_FEATURE (1)..(1): Xaa in position 1 is N-term (-NH2) A, L, I, or V
  MISC_FEATURE (2)..(2): Xaa in position 2 is S, T, G, A, N, E or D
  MISC_FEATURE (3)..(3): Xaa in position 3 is D, E, or G
  MISC_FEATURE (5)..(5): Xaa in position 5 is P, N, S, D, A, T, K, or G
  MISC_FEATURE (6)..(6): Xaa in position 6 is Y, N, I, W, or F
  MISC_FEATURE (7)..(7): Xaa in position 7 is I, L, R, or V
  MISC_FEATURE (8)..(8): Xaa in position 8 is a C-term L, I, V, S, M, or T
XXXKXXXX

SEQ ID NO: 3 - protein, 8 aa, Artificial Sequence
  Artificial peptide sequence
  MISC_FEATURE (1)..(1): Xaa in position 1 is A, L, I, or V
  MISC_FEATURE (2)..(2): Xaa in position 2 is S, T, G, A, N, E or D
  MISC_FEATURE (3)..(3): Xaa in position 3 is D, R, K, E, or G
  MISC_FEATURE (4)..(4): Xaa in position 4 is K or R
  MISC_FEATURE (5)..(5): Xaa in position 5 is P, N, S, D, A, T, K, or G
  MISC_FEATURE (6)..(6): Xaa in position 6 is Y, N, I, W, or F
  MISC_FEATURE (7)..(7): Xaa in position 7 is I, L, R, or V
  MISC_FEATURE (8)..(8): Xaa in position 8 is L, I, V, S, M, or T
XXXXXXXX

SEQ ID NO: 4 - protein, 4 aa, Artificial Sequence
  Artificial peptide sequence
PYIL

SEQ ID NO: 5 - protein, 16 aa, Artificial Sequence
  Artificial peptide sequence
AVTEKKYILYDFSVTS

SEQ ID NO: 6 - protein, 8 aa, Artificial Sequence
  Artificial peptide sequence
ASDKPYIL

SEQ ID NO: 7 - protein, 7 aa, Artificial Sequence
  Artificial peptide sequence
SDKPYIL

SEQ ID NO: 8 - protein, 6 aa, Artificial Sequence
  Artificial peptide sequence
DKPYIL

SEQ ID NO: 9 - protein, 5 aa, Artificial Sequence
  Artificial peptide sequence
KPYIL

SEQ ID NO: 10 - protein, 8 aa, Artificial Sequence
  Artificial peptide sequence
AGDKNYIL

SEQ ID NO: 11 - protein, 8 aa, Artificial Sequence
  Artificial peptide sequence
AGDKNYIT

SEQ ID NO: 12 - protein, 8 aa, Artificial Sequence
  Artificial peptide sequence
AGDKSYIT

SEQ ID NO: 13 - protein, 8 aa, Artificial Sequence
  Artificial peptide sequence
ADGKPYIV

SEQ ID NO: 14 - protein, 8 aa, Artificial Sequence
  Artificial peptide sequence
AEDKDFIT

SEQ ID NO: 15 - protein, 8 aa, Artificial Sequence
  Artificial peptide sequence
AADKPYIL

SEQ ID NO: 16 - protein, 8 aa, Artificial Sequence
  Artificial peptide sequence
ATDKPYIL

SEQ ID NO: 17 - protein, 8 aa, Artificial Sequence
  Artificial peptide sequence
AGDKPYIT

SEQ ID NO: 18 - protein, 8 aa, Artificial Sequence
  Artificial peptide sequence
ASEKPYIL

SEQ ID NO: 19 - protein, 8 aa, Artificial Sequence
  Artificial peptide sequence
ADGKPYVT

SEQ ID NO: 20 - protein, 8 aa, Artificial Sequence
  Artificial peptide sequence
AGDKPYIL

SEQ ID NO: 21 - protein, 8 aa, Artificial Sequence
  Artificial peptide sequence
ASDKPNIL

SEQ ID NO: 22 - protein, 8 aa, Artificial Sequence
  Artificial peptide sequence
ASDKPYIT

SEQ ID NO: 23 - protein, 8 aa, Artificial Sequence
  Artificial peptide sequence
AADKPFIL

SEQ ID NO: 24 - protein, 8 aa, Artificial Sequence
  Artificial peptide sequence
ASDKAYIT

SEQ ID NO: 25 - protein, 8 aa, Artificial Sequence
  Artificial peptide sequence
AGDKAYIT

SEQ ID NO: 26 - protein, 8 aa, Artificial Sequence
  Artificial peptide sequence
ANGKPFIT

SEQ ID NO: 27 - protein, 8 aa, Artificial Sequence
  Artificial peptide sequence
AGDKNFIT

SEQ ID NO: 28 - protein, 8 aa, Artificial Sequence
  Artificial peptide sequence
ASDKSYIT

SEQ ID NO: 29 - protein, 8 aa, Artificial Sequence
  Artificial peptide sequence
ASDKTYIT

SEQ ID NO: 30 - protein, 8 aa, Artificial Sequence
  Artificial peptide sequence
ASDKNYIT

SEQ ID NO: 31 - protein, 8 aa, Artificial Sequence
  Artificial peptide sequence
AGDKKYIT

SEQ ID NO: 32 - protein, 8 aa, Artificial Sequence
  Artificial peptide sequence
AGDKNYIS

SEQ ID NO: 33 - protein, 8 aa, Artificial Sequence
  Artificial peptide sequence
AADKNYIT

SEQ ID NO: 34 - protein, 8 aa, Artificial Sequence
  Artificial peptide sequence
AGDKNYIM

SEQ ID NO: 35 - protein, 8 aa, Artificial Sequence
  Artificial peptide sequence
AADKNFIM

SEQ ID NO: 36 - protein, 8 aa, Artificial Sequence
  Artificial peptide sequence
AADKNFIT

SEQ ID NO: 37 - protein, 8 aa, Artificial Sequence
  Artificial peptide sequence
AGDKGIRS

SEQ ID NO: 38 - protein, 7 aa, Artificial Sequence
  Artificial peptide sequence
PRRPYIL

SEQ ID NO: 39 - protein, 6 aa, Artificial Sequence
  Artificial peptide sequence
RRPYIL

SEQ ID NO: 40 - protein, 5 aa, Artificial Sequence
  Artificial peptide sequence
RPYIL

SEQ ID NO: 41 - protein, 6 aa, Artificial Sequence
  Artificial peptide sequence
RRPWIL

SEQ ID NO: 42 - protein, 6 aa, Artificial Sequence
  Artificial peptide sequence
KRPYIL

SEQ ID NO: 43 - protein, 6 aa, Artificial Sequence
  Artificial peptide sequence
KKPYIL

SEQ ID NO: 44 - protein, 6 aa, Artificial Sequence
  Artificial peptide sequence
  misc_feature (2)..(2): Xaa can be any naturally occurring amino acid
KXPYIL

SEQ ID NO: 45 - protein, 5 aa, Artificial Sequence
  Artificial peptide sequence
KPYII

SEQ ID NO: 46 - protein, 5 aa, Artificial Sequence
  Artificial peptide sequence
KPYIV

SEQ ID NO: 47 - protein, 5 aa, Artificial Sequence
  Artificial peptide sequence
KPYLL

SEQ ID NO: 48 - protein, 5 aa, Artificial Sequence
  Artificial peptide sequence
KPYLI

SEQ ID NO: 49 - protein, 5 aa, Artificial Sequence
  Artificial peptide sequence
KPYLV

SEQ ID NO: 50 - protein, 5 aa, Artificial Sequence
  Artificial peptide sequence
KPYVL

SEQ ID NO: 51 - protein, 5 aa, Artificial Sequence
  Artificial peptide sequence
KPYVI

SEQ ID NO: 52 - protein, 5 aa, Artificial Sequence
  Artificial peptide sequence
KPYVV

SEQ ID NO: 53 - protein, 5 aa, Artificial Sequence
  Artificial peptide sequence
KPWIL

SEQ ID NO: 54 - protein, 5 aa, Artificial Sequence
  Artificial peptide sequence
KPWII

SEQ ID NO: 55 - protein, 5 aa, Artificial Sequence
  Artificial peptide sequence
KPWIV

SEQ ID NO: 56 - protein, 5 aa, Artificial Sequence
  Artificial peptide sequence
KPWLL

SEQ ID NO: 57 - protein, 5 aa, Artificial Sequence
  Artificial peptide sequence
KPWLI

SEQ ID NO: 58 - protein, 5 aa, Artificial Sequence
  Artificial peptide sequence
KPWLV

SEQ ID NO: 59 - protein, 5 aa, Artificial Sequence
  Artificial peptide sequence
KPWVL

SEQ ID NO: 60 - protein, 5 aa, Artificial Sequence
  Artificial peptide sequence
KPWVI

SEQ ID NO: 61 - protein, 5 aa, Artificial Sequence
  Artificial peptide sequence
KPWVV

SEQ ID NO: 62 - protein, 5 aa, Artificial Sequence
  Artificial peptide sequence
RPYII

SEQ ID NO: 63 - protein, 5 aa, Artificial Sequence
  Artificial peptide sequence
RPYIV

SEQ ID NO: 64 - protein, 5 aa, Artificial Sequence
  Artificial peptide sequence
RPYLL

SEQ ID NO: 65 - protein, 5 aa, Artificial Sequence
  Artificial peptide sequence
RPYLI

SEQ ID NO: 66 - protein, 5 aa, Artificial Sequence
  Artificial peptide sequence
RPYLV

SEQ ID NO: 67 - protein, 5 aa, Artificial Sequence
  Artificial peptide sequence
RPYVL

SEQ ID NO: 68 - protein, 5 aa, Artificial Sequence
  Artificial peptide sequence
RPYVI

SEQ ID NO: 69 - protein, 5 aa, Artificial Sequence
  Artificial peptide sequence
RPYVV

SEQ ID NO: 70 - protein, 5 aa, Artificial Sequence
  Artificial peptide sequence
RPWIL

SEQ ID NO: 71 - protein, 5 aa, Artificial Sequence
  Artificial peptide sequence
RPWII

SEQ ID NO: 72 - protein, 5 aa, Artificial Sequence
  Artificial peptide sequence
RPWIV

SEQ ID NO: 73 - protein, 5 aa, Artificial Sequence
  Artificial peptide sequence
RPWLL

SEQ ID NO: 74 - protein, 5 aa, Artificial Sequence
  Artificial peptide sequence
RPWLI

SEQ ID NO: 75 - protein, 5 aa, Artificial Sequence
  Artificial peptide sequence
RPWLV

SEQ ID NO: 76 - protein, 5 aa, Artificial Sequence
  Artificial peptide sequence
RPWVL

SEQ ID NO: 77 - protein, 5 aa, Artificial Sequence
  Artificial peptide sequence
RPWVI

SEQ ID NO: 78 - protein, 5 aa, Artificial Sequence
  Artificial peptide sequence
RPWVV

SEQ ID NO: 79 - protein, 6 aa, Artificial Sequence
  Artificial peptide sequence
DKPYII

SEQ ID NO: 80 - protein, 6 aa, Artificial Sequence
  Artificial peptide sequence
DKPYIV

SEQ ID NO: 81 - protein, 6 aa, Artificial Sequence
  Artificial peptide sequence
DKPYLL

SEQ ID NO: 82 - protein, 6 aa, Artificial Sequence
  Artificial peptide sequence
DKPYLI

SEQ ID NO: 83 - protein, 6 aa, Artificial Sequence
  Artificial peptide sequence
DKPYLV

SEQ ID NO: 84 - protein, 6 aa, Artificial Sequence
  Artificial peptide sequence
DKPYVL

SEQ ID NO: 85 - protein, 6 aa, Artificial Sequence
  Artificial peptide sequence
DKPYVI

SEQ ID NO: 86 - protein, 6 aa, Artificial Sequence
  Artificial peptide sequence
DKPYVV

SEQ ID NO: 87 - protein, 6 aa, Artificial Sequence
  Artificial peptide sequence
DKPWIL

SEQ ID NO: 88 - protein, 6 aa, Artificial Sequence
  Artificial peptide sequence
DKPWII

SEQ ID NO: 89 - protein, 6 aa, Artificial Sequence
  Artificial peptide sequence
DKPWIV

SEQ ID NO: 90 - protein, 6 aa, Artificial Sequence
  Artificial peptide sequence
DKPWLL

SEQ ID NO: 91 - protein, 6 aa, Artificial Sequence
  Artificial peptide sequence
DKPWLI

SEQ ID NO: 92 - protein, 6 aa, Artificial Sequence
  Artificial peptide sequence
DKPWLV

SEQ ID NO: 93 - protein, 6 aa, Artificial Sequence
  Artificial peptide sequence
DKPWVL

SEQ ID NO: 94 - protein, 6 aa, Artificial Sequence
  Artificial peptide sequence
DKPWVI

SEQ ID NO: 95 - protein, 6 aa, Artificial Sequence
  Artificial peptide sequence
DKPWVV

SEQ ID NO: 96 - protein, 6 aa, Artificial Sequence
  Artificial peptide sequence
DRPYIL

SEQ ID NO: 97 - protein, 6 aa, Artificial Sequence
  Artificial peptide sequence
DRPYII

SEQ ID NO: 98 - protein, 6 aa, Artificial Sequence
  Artificial peptide sequence
DRPYIV

SEQ ID NO: 99 - protein, 6 aa, Artificial Sequence
  Artificial peptide sequence
DRPYLL

SEQ ID NO: 100 - protein, 6 aa, Artificial Sequence
  Artificial peptide sequence
DRPYLI

SEQ ID NO: 101 - protein, 6 aa, Artificial Sequence
  Artificial peptide sequence
DRPYLV

SEQ ID NO: 102 - protein, 6 aa, Artificial Sequence
  Artificial peptide sequence
DRPYVL

SEQ ID NO: 103 - protein, 6 aa, Artificial Sequence
  Artificial peptide sequence
DRPYVI

SEQ ID NO: 104 - protein, 6 aa, Artificial Sequence
  Artificial peptide sequence
DRPYVV

SEQ ID NO: 105 - protein, 6 aa, Artificial Sequence
  Artificial peptide sequence
DRPWIL

SEQ ID NO: 106 - protein, 6 aa, Artificial Sequence
  Artificial peptide sequence
DRPWII

SEQ ID NO: 107 - protein, 6 aa, Artificial Sequence
  Artificial peptide sequence
DRPWIV

SEQ ID NO: 108 - protein, 6 aa, Artificial Sequence
  Artificial peptide sequence
DRPWLL

SEQ ID NO: 109 - protein, 6 aa, Artificial Sequence
  Artificial peptide sequence
DRPWLI

SEQ ID NO: 110 - protein, 6 aa, Artificial Sequence
  Artificial peptide sequence
DRPWLV

SEQ ID NO: 111 - protein, 6 aa, Artificial Sequence
  Artificial peptide sequence
DRPWVL

SEQ ID NO: 112 - protein, 6 aa, Artificial Sequence
  Artificial peptide sequence
DRPWVI

SEQ ID NO: 113 - protein, 6 aa, Artificial Sequence
  Artificial peptide sequence
DRPWVV

SEQ ID NO: 114 - protein, 6 aa, Artificial Sequence
  Artificial peptide sequence
EKPYIL

SEQ ID NO: 115 - protein, 6 aa, Artificial Sequence
  Artificial peptide sequence
EKPYII

SEQ ID NO: 116 - protein, 6 aa, Artificial Sequence
  Artificial peptide sequence
EKPYIV

SEQ ID NO: 117 - protein, 6 aa, Artificial Sequence
  Artificial peptide sequence
EKPYLL

SEQ ID NO: 118 - protein, 6 aa, Artificial Sequence
  Artificial peptide sequence
EKPYLI

SEQ ID NO: 119 - protein, 6 aa, Artificial Sequence
  Artificial peptide sequence
EKPYLV

SEQ ID NO: 120 - protein, 6 aa, Artificial Sequence
  Artificial peptide sequence
EKPYVL

SEQ ID NO: 121 - protein, 6 aa, Artificial Sequence
  Artificial peptide sequence
EKPYVI

SEQ ID NO: 122 - protein, 6 aa, Artificial Sequence
  Artificial peptide sequence
EKPYVV

SEQ ID NO: 123 - protein, 6 aa, Artificial Sequence
  Artificial peptide sequence
EKPWIL

SEQ ID NO: 124 - protein, 6 aa, Artificial Sequence
  Artificial peptide sequence
EKPWII

SEQ ID NO: 125 - protein, 6 aa, Artificial Sequence
  Artificial peptide sequence
EKPWIV

SEQ ID NO: 126 - protein, 6 aa, Artificial Sequence
  Artificial peptide sequence
EKPWLL

SEQ ID NO: 127 - protein, 6 aa, Artificial Sequence
  Artificial peptide sequence
EKPWLI

SEQ ID NO: 128 - protein, 6 aa, Artificial Sequence
  Artificial peptide sequence
EKPWLV

SEQ ID NO: 129 - protein, 6 aa, Artificial Sequence
  Artificial peptide sequence
EKPWVL

SEQ ID NO: 130 - protein, 6 aa, Artificial Sequence
  Artificial peptide sequence
EKPWVI

SEQ ID NO: 131 - protein, 6 aa, Artificial Sequence
  Artificial peptide sequence
EKPWVV

SEQ ID NO: 132 - protein, 6 aa, Artificial Sequence
  Artificial peptide sequence
ERPYIL

SEQ ID NO: 133 - protein, 6 aa, Artificial Sequence
  Artificial peptide sequence
ERPYII

SEQ ID NO: 134 - protein, 6 aa, Artificial Sequence
  Artificial peptide sequence
ERPYIV

SEQ ID NO: 135 - protein, 6 aa, Artificial Sequence
  Artificial peptide sequence
ERPYLL

SEQ ID NO: 136 - protein, 6 aa, Artificial Sequence
  Artificial peptide sequence
ERPYLI

SEQ ID NO: 137 - protein, 6 aa, Artificial Sequence
  Artificial peptide sequence
ERPYLV

SEQ ID NO: 138 - protein, 6 aa, Artificial Sequence
  Artificial peptide sequence
ERPYVL

SEQ ID NO: 139 - protein, 6 aa, Artificial Sequence
  Artificial peptide sequence
ERPYVI

SEQ ID NO: 140 - protein, 6 aa, Artificial Sequence
  Artificial peptide sequence
ERPYVV

SEQ ID NO: 141 - protein, 6 aa, Artificial Sequence
  Artificial peptide sequence
ERPWIL

SEQ ID NO: 142 - protein, 6 aa, Artificial Sequence
  Artificial peptide sequence
ERPWII

SEQ ID NO: 143 - protein, 6 aa, Artificial Sequence
  Artificial peptide sequence
ERPWIV

SEQ ID NO: 144 - protein, 6 aa, Artificial Sequence
  Artificial peptide sequence
ERPWLL

SEQ ID NO: 145 - protein, 6 aa, Artificial Sequence
  Artificial peptide sequence
ERPWLI

SEQ ID NO: 146 - protein, 6 aa, Artificial Sequence
  Artificial peptide sequence
ERPWLV

SEQ ID NO: 147 - protein, 6 aa, Artificial Sequence
  Artificial peptide sequence
ERPWVL

SEQ ID NO: 148 - protein, 6 aa, Artificial Sequence
  Artificial peptide sequence
ERPWVI

SEQ ID NO: 149 - protein, 6 aa, Artificial Sequence
  Artificial peptide sequence
ERPWVV

SEQ ID NO: 150 - protein, 6 aa, Artificial Sequence
  Artificial peptide sequence
RKPYIL

SEQ ID NO: 151 - protein, 6 aa, Artificial Sequence
  Artificial peptide sequence
RKPYII

SEQ ID NO: 152 - protein, 6 aa, Artificial Sequence
  Artificial peptide sequence
RKPYIV

SEQ ID NO: 153 - protein, 6 aa, Artificial Sequence
  Artificial peptide sequence
RKPYLL

SEQ ID NO: 154 - protein, 6 aa, Artificial Sequence
  Artificial peptide sequence
RKPYLI

SEQ ID NO: 155 - protein, 6 aa, Artificial Sequence
  Artificial peptide sequence
RKPYLV

SEQ ID NO: 156 - protein, 6 aa, Artificial Sequence
  Artificial peptide sequence
RKPYVL

SEQ ID NO: 157 - protein, 6 aa, Artificial Sequence
  Artificial peptide sequence
RKPYVI

SEQ ID NO: 158 - protein, 6 aa, Artificial Sequence
  Artificial peptide sequence
RKPYVV

SEQ ID NO: 159 - protein, 6 aa, Artificial Sequence
  Artificial peptide sequence
RKPWIL

SEQ ID NO: 160 - protein, 6 aa, Artificial Sequence
  Artificial peptide sequence
RKPWII

SEQ ID NO: 161 - protein, 6 aa, Artificial Sequence
  Artificial peptide sequence
RKPWIV

SEQ ID NO: 162 - protein, 6 aa, Artificial Sequence
  Artificial peptide sequence
RKPWLL

SEQ ID NO: 163 - protein, 6 aa, Artificial Sequence
  Artificial peptide sequence
RKPWLI

SEQ ID NO: 164 - protein, 6 aa, Artificial Sequence
  Artificial peptide sequence
RKPWLV

SEQ ID NO: 165 - protein, 6 aa, Artificial Sequence
  Artificial peptide sequence
RKPWVL

SEQ ID NO: 166 - protein, 6 aa, Artificial Sequence
  Artificial peptide sequence
RKPWVI

SEQ ID NO: 167 - protein, 6 aa, Artificial Sequence
  Artificial peptide sequence
RKPWVV

SEQ ID NO: 168 - protein, 6 aa, Artificial Sequence
  Artificial peptide sequence
RRPYII

SEQ ID NO: 169 - protein, 6 aa, Artificial Sequence
  Artificial peptide sequence
RRPYIV

SEQ ID NO: 170 - protein, 6 aa, Artificial Sequence
  Artificial peptide sequence
RRPYLL

SEQ ID NO: 171 - protein, 6 aa, Artificial Sequence
  Artificial peptide sequence
RRPYLI

SEQ ID NO: 172 - protein, 6 aa, Artificial Sequence
  Artificial peptide sequence
RRPYLV

SEQ ID NO: 173 - protein, 6 aa, Artificial Sequence
  Artificial peptide sequence
RRPYVL

SEQ ID NO: 174 - protein, 6 aa, Artificial Sequence
  Artificial peptide sequence
RRPYVI

SEQ ID NO: 175 - protein, 6 aa, Artificial Sequence
  Artificial peptide sequence
RRPYVV

SEQ ID NO: 176 - protein, 6 aa, Artificial Sequence
  Artificial peptide sequence
RRPWII

SEQ ID NO: 177 - protein, 6 aa, Artificial Sequence
  Artificial peptide sequence
RRPWIV

SEQ ID NO: 178 - protein, 6 aa, Artificial Sequence
  Artificial peptide sequence
RRPWLL

SEQ ID NO: 179 - protein, 6 aa, Artificial Sequence
  Artificial peptide sequence
RRPWLI

SEQ ID NO: 180 - protein, 6 aa, Artificial Sequence
  Artificial peptide sequence
RRPWLV

SEQ ID NO: 181 - protein, 6 aa, Artificial Sequence
  Artificial peptide sequence
RRPWVL

SEQ ID NO: 182 - protein, 6 aa, Artificial Sequence
  Artificial peptide sequence
RRPWVI

SEQ ID NO: 183 - protein, 6 aa, Artificial Sequence
  Artificial peptide sequence
RRPWVV

SEQ ID NO: 184 - protein, 6 aa, Artificial Sequence
  Artificial peptide sequence
GKPYIL

SEQ ID NO: 185 - protein, 6 aa, Artificial Sequence
  Artificial peptide sequence
GKPYII

SEQ ID NO: 186 - protein, 6 aa, Artificial Sequence
  Artificial peptide sequence
GKPYIV

SEQ ID NO: 187 - protein, 6 aa, Artificial Sequence
  Artificial peptide sequence
GKPYLL

SEQ ID NO: 188 - protein, 6 aa, Artificial Sequence
  Artificial peptide sequence
GKPYLI

SEQ ID NO: 189 - protein, 6 aa, Artificial Sequence
  Artificial peptide sequence
GKPYLV

SEQ ID NO: 190 - protein, 6 aa, Artificial Sequence
  Artificial peptide sequence
GKPYVL

SEQ ID NO: 191 - protein, 6 aa, Artificial Sequence
  Artificial peptide sequence
GKPYVI

SEQ ID NO: 192 - protein, 6 aa, Artificial Sequence
  Artificial peptide sequence
GKPYVV

SEQ ID NO: 193 - protein, 6 aa, Artificial Sequence
  Artificial peptide sequence
GKPWIL

SEQ ID NO: 194 - protein, 6 aa, Artificial Sequence
  Artificial peptide sequence
GKPWII

SEQ ID NO: 195 - protein, 6 aa, Artificial Sequence
  Artificial peptide sequence
GKPWIV

SEQ ID NO: 196 - protein, 6 aa, Artificial Sequence
  Artificial peptide sequence
GKPWLL

SEQ ID NO: 197 - protein, 6 aa, Artificial Sequence
  Artificial peptide sequence
GKPWLI

SEQ ID NO: 198 - protein, 6 aa, Artificial Sequence
  Artificial peptide sequence
GKPWLV

SEQ ID NO: 199 - protein, 6 aa, Artificial Sequence
  Artificial peptide sequence
GKPWVL

SEQ ID NO: 200 - protein, 6 aa, Artificial Sequence
  Artificial peptide sequence
GKPWVI

SEQ ID NO: 201 - protein, 6 aa, Artificial Sequence
  Artificial peptide sequence
GKPWVV

SEQ ID NO: 202 - protein, 6 aa, Artificial Sequence
  Artificial peptide sequence
GRPYIL

SEQ ID NO: 203 - protein, 6 aa, Artificial Sequence
  Artificial peptide sequence
GRPYII

SEQ ID NO: 204 - protein, 6 aa, Artificial Sequence
  Artificial peptide sequence
GRPYIV

SEQ ID NO: 205 - protein, 6 aa, Artificial Sequence
  Artificial peptide sequence
GRPYLL

SEQ ID NO: 206 - protein, 6 aa, Artificial Sequence
  Artificial peptide sequence
GRPYLI

SEQ ID NO: 207 - protein, 6 aa, Artificial Sequence
  Artificial peptide sequence
GRPYLV

SEQ ID NO: 208 - protein, 6 aa, Artificial Sequence
  Artificial peptide sequence
GRPYVL

SEQ ID NO: 209 - protein, 6 aa, Artificial Sequence
  Artificial peptide sequence
GRPYVI

SEQ ID NO: 210 - protein, 6 aa, Artificial Sequence
  Artificial peptide sequence
GRPYVV

SEQ ID NO: 211 - protein, 6 aa, Artificial Sequence
  Artificial peptide sequence
GRPWIL

SEQ ID NO: 212 - protein, 6 aa, Artificial Sequence
  Artificial peptide sequence
GRPWII

SEQ ID NO: 213 - protein, 6 aa, Artificial Sequence
  Artificial peptide sequence
GRPWIV

SEQ ID NO: 214 - protein, 6 aa, Artificial Sequence
  Artificial peptide sequence
GRPWLL

SEQ ID NO: 215 - protein, 6 aa, Artificial Sequence
  Artificial peptide sequence
GRPWLI

SEQ ID NO: 216 - protein, 6 aa, Artificial Sequence
  Artificial peptide sequence
GRPWLV

SEQ ID NO: 217 - protein, 6 aa, Artificial Sequence
  Artificial peptide sequence
GRPWVL

SEQ ID NO: 218 - protein, 6 aa, Artificial Sequence
  Artificial peptide sequence
GRPWVI

SEQ ID NO: 219 - protein, 6 aa, Artificial Sequence
  Artificial peptide sequence
GRPWVV

SEQ ID NO: 220 - protein, 7 aa, Artificial Sequence
  Artificial peptide sequence
SDKPYIL

SEQ ID NO: 221 - protein, 7 aa, Artificial Sequence
  Artificial peptide sequence
SDKPYII

SEQ ID NO: 222 - protein, 7 aa, Artificial Sequence
  Artificial peptide sequence
SDKPYIV

SEQ ID NO: 223 - protein, 7 aa, Artificial Sequence
  Artificial peptide sequence
SDKPYLL

SEQ ID NO: 224 - protein, 7 aa, Artificial Sequence
  Artificial peptide sequence
SDKPYLI

SEQ ID NO: 225 - protein, 7 aa, Artificial Sequence
  Artificial peptide sequence
SDKPYLV

SEQ ID NO: 226 - protein, 7 aa, Artificial Sequence
  Artificial peptide sequence
SDKPYVL

SEQ ID NO: 227 - protein, 7 aa, Artificial Sequence
  Artificial peptide sequence
SDKPYVI

SEQ ID NO: 228 - protein, 7 aa, Artificial Sequence
  Artificial peptide sequence
SDKPYVV

SEQ ID NO: 229 - protein, 7 aa, Artificial Sequence
  Artificial peptide sequence
SDKPWIL

SEQ ID NO: 230 - protein, 7 aa, Artificial Sequence
  Artificial peptide sequence
SDKPWII

SEQ ID NO: 231 - protein, 7 aa, Artificial Sequence
  Artificial peptide sequence
SDKPWIV

SEQ ID NO: 232 - protein, 7 aa, Artificial Sequence
  Artificial peptide sequence
SDKPWLL

SEQ ID NO: 233 - protein, 7 aa, Artificial Sequence
  Artificial peptide sequence
SDKPWLI

SEQ ID NO: 234 - protein, 7 aa, Artificial Sequence
  Artificial peptide sequence
SDKPWLV

SEQ ID NO: 235 - protein, 7 aa, Artificial Sequence
  Artificial peptide sequence
SDKPWVL

SEQ ID NO: 236 - protein, 7 aa, Artificial Sequence
  Artificial peptide sequence
SDKPWVI

SEQ ID NO: 237 - protein, 7 aa, Artificial Sequence
  Artificial peptide sequence
SDKPWVV

SEQ ID NO: 238 - protein, 7 aa, Artificial Sequence
  Artificial peptide sequence
SDRPYIL

SEQ ID NO: 239 - protein, 7 aa, Artificial Sequence
  Artificial peptide sequence
SDRPYII

SEQ ID NO: 240 - protein, 7 aa, Artificial Sequence
  Artificial peptide sequence
SDRPYIV

SEQ ID NO: 241 - protein, 7 aa, Artificial Sequence
  Artificial peptide sequence
SDRPYLL

SEQ ID NO: 242 - protein, 7 aa, Artificial Sequence
  Artificial peptide sequence
SDRPYLI

SEQ ID NO: 243 - protein, 7 aa, Artificial Sequence
  Artificial peptide sequence
SDRPYLV

SEQ ID NO: 244 - protein, 7 aa, Artificial Sequence
  Artificial peptide sequence
SDRPYVL

SEQ ID NO: 245 - protein, 7 aa, Artificial Sequence
  Artificial peptide sequence
SDRPYVI

SEQ ID NO: 246 - protein, 7 aa, Artificial Sequence
  Artificial peptide sequence
SDRPYVV

SEQ ID NO: 247 - protein, 7 aa, Artificial Sequence
  Artificial peptide sequence
SDRPWIL

SEQ ID NO: 248 - protein, 7 aa, Artificial Sequence
  Artificial peptide sequence
SDRPWII

SEQ ID NO: 249 - protein, 7 aa, Artificial Sequence
  Artificial peptide sequence
SDRPWIV

SEQ ID NO: 250 - protein, 7 aa, Artificial Sequence
  Artificial peptide sequence
SDRPWLL

SEQ ID NO: 251 - protein, 7 aa, Artificial Sequence
  Artificial peptide sequence
SDRPWLI

SEQ ID NO: 252 - protein, 7 aa, Artificial Sequence
  Artificial peptide sequence
SDRPWLV

SEQ ID NO: 253 - protein, 7 aa, Artificial Sequence
  Artificial peptide sequence
SDRPWVL

SEQ ID NO: 254 - protein, 7 aa, Artificial Sequence
  Artificial peptide sequence
SDRPWVI

SEQ ID NO: 255 - protein, 7 aa, Artificial Sequence
  Artificial peptide sequence
SDRPWVV

SEQ ID NO: 256 - protein, 7 aa, Artificial Sequence
  Artificial peptide sequence
SEKPYIL

SEQ ID NO: 257 - protein, 7 aa, Artificial Sequence
  Artificial peptide sequence
SEKPYII

SEQ ID NO: 258 - protein, 7 aa, Artificial Sequence
  Artificial peptide sequence
SEKPYIV

SEQ ID NO: 259 - protein, 7 aa, Artificial Sequence
  Artificial peptide sequence
SEKPYLL

SEQ ID NO: 260 - protein, 7 aa, Artificial Sequence
  Artificial peptide sequence
SEKPYLI

SEQ ID NO: 261 - protein, 7 aa, Artificial Sequence
  Artificial peptide sequence
SEKPYLV

SEQ ID NO: 262 - protein, 7 aa, Artificial Sequence
  Artificial peptide sequence
SEKPYVL

SEQ ID NO: 263 - protein, 7 aa, Artificial Sequence
  Artificial peptide sequence
SEKPYVI

SEQ ID NO: 264 - protein, 7 aa, Artificial Sequence
  Artificial peptide sequence
SEKPYVV

SEQ ID NO: 265 - protein, 7 aa, Artificial Sequence
  Artificial peptide sequence
SEKPWIL

SEQ ID NO: 266 - protein, 7 aa, Artificial Sequence
  Artificial peptide sequence
SEKPWII

SEQ ID NO: 267 - protein, 7 aa, Artificial Sequence
  Artificial peptide sequence
SEKPWIV

SEQ ID NO: 268 - protein, 7 aa, Artificial Sequence
  Artificial peptide sequence
SEKPWLL

SEQ ID NO: 269 - protein, 7 aa, Artificial Sequence
  Artificial peptide sequence
SEKPWLI

SEQ ID NO: 270 - protein, 7 aa, Artificial Sequence
  Artificial peptide sequence
SEKPWLV

SEQ ID NO: 271 - protein, 7 aa, Artificial Sequence
  Artificial peptide sequence
SEKPWVL

SEQ ID NO: 272 - protein, 7 aa, Artificial Sequence
  Artificial peptide sequence
SEKPWVI

SEQ ID NO: 273 - protein, 7 aa, Artificial Sequence
  Artificial peptide sequence
SEKPWVV

SEQ ID NO: 274 - protein, 7 aa, Artificial Sequence
  Artificial peptide sequence
SERPYIL

SEQ ID NO: 275 - protein, 7 aa, Artificial Sequence
  Artificial peptide sequence
SERPYII

SEQ ID NO: 276 - protein, 7 aa, Artificial Sequence
  Artificial peptide sequence
SERPYIV

SEQ ID NO: 277 - protein, 7 aa, Artificial Sequence
  Artificial peptide sequence
SERPYLL

SEQ ID NO: 278 - protein, 7 aa, Artificial Sequence
  Artificial peptide sequence
SERPYLI

SEQ ID NO: 279 - protein, 7 aa, Artificial Sequence
  Artificial peptide sequence
SERPYLV

SEQ ID NO: 280 - protein, 7 aa, Artificial Sequence
  Artificial peptide sequence
SERPYVL

SEQ ID NO: 281 - protein, 7 aa, Artificial Sequence
  Artificial peptide sequence
SERPYVI

SEQ ID NO: 282 - protein, 7 aa, Artificial Sequence
  Artificial peptide sequence
SERPYVV

SEQ ID NO: 283 - protein, 7 aa, Artificial Sequence
  Artificial peptide sequence
SERPWIL

SEQ ID NO: 284 - protein, 7 aa, Artificial Sequence
  Artificial peptide sequence
SERPWII

SEQ ID NO: 285 - protein, 7 aa, Artificial Sequence
  Artificial peptide sequence
SERPWIV

SEQ ID NO: 286 - protein, 7 aa, Artificial Sequence
  Artificial peptide sequence
SERPWLL

SEQ ID NO: 287 - protein, 7 aa, Artificial Sequence
  Artificial peptide sequence
SERPWLI

SEQ ID NO: 288 - protein, 7 aa, Artificial Sequence
  Artificial peptide sequence
SERPWLV

SEQ ID NO: 289 - protein, 7 aa, Artificial Sequence
  Artificial peptide sequence
SERPWVL

SEQ ID NO: 290 - protein, 7 aa, Artificial Sequence
  Artificial peptide sequence
SERPWVI

SEQ ID NO: 291 - protein, 7 aa, Artificial Sequence
  Artificial peptide sequence
SERPWVV

SEQ ID NO: 292 - protein, 7 aa, Artificial Sequence
  Artificial peptide sequence
TDKPYIL

SEQ ID NO: 293 - protein, 7 aa, Artificial Sequence
  Artificial peptide sequence
TDKPYII

SEQ ID NO: 294 - protein, 7 aa, Artificial Sequence
  Artificial peptide sequence
TDKPYIV

SEQ ID NO: 295 - protein, 7 aa, Artificial Sequence
  Artificial peptide sequence
TDKPYLL

SEQ ID NO: 296 - protein, 7 aa, Artificial Sequence
  Artificial peptide sequence
TDKPYLI

SEQ ID NO: 297 - protein, 7 aa, Artificial Sequence
  Artificial peptide sequence
TDKPYLV

SEQ ID NO: 298 - protein, 7 aa, Artificial Sequence
  Artificial peptide sequence
TDKPYVL

SEQ ID NO: 299 - protein, 7 aa, Artificial Sequence
  Artificial peptide sequence
TDKPYVI

SEQ ID NO: 300 - protein, 7 aa, Artificial Sequence
  Artificial peptide sequence
TDKPYVV

SEQ ID NO: 301 - protein, 7 aa, Artificial Sequence
  Artificial peptide sequence
TDKPWIL

SEQ ID NO: 302 - protein, 7 aa, Artificial Sequence
  Artificial peptide sequence
TDKPWII

SEQ ID NO: 303 - protein, 7 aa, Artificial Sequence
  Artificial peptide sequence
TDKPWIV

SEQ ID NO: 304 - protein, 7 aa, Artificial Sequence
  Artificial peptide sequence
TDKPWLL

SEQ ID NO: 305 - protein, 7 aa, Artificial Sequence
  Artificial peptide sequence
TDKPWLI

SEQ ID NO: 306 - protein, 7 aa, Artificial Sequence
  Artificial peptide sequence
TDKPWLV

SEQ ID NO: 307 - protein, 7 aa, Artificial Sequence
  Artificial peptide sequence
TDKPWVL

SEQ ID NO: 308 - protein, 7 aa, Artificial Sequence
  Artificial peptide sequence
TDKPWVI

SEQ ID NO: 309 - protein, 7 aa, Artificial Sequence
  Artificial peptide sequence
TDKPWVV

SEQ ID NO: 310 - protein, 7 aa, Artificial Sequence
  Artificial peptide sequence
TDRPYIL

SEQ ID NO: 311 - protein, 7 aa, Artificial Sequence
  Artificial peptide sequence
TDRPYII

SEQ ID NO: 312 - protein, 7 aa, Artificial Sequence
  Artificial peptide sequence
TDRPYIV

SEQ ID NO: 313 - protein, 7 aa, Artificial Sequence
  Artificial peptide sequence
TDRPYLL

SEQ ID NO: 314 - protein, 7 aa, Artificial Sequence
  Artificial peptide sequence
TDRPYLI

SEQ ID NO: 315 - protein, 7 aa, Artificial Sequence
  Artificial peptide sequence
TDRPYLV

SEQ ID NO: 316 - protein, 7 aa, Artificial Sequence
  Artificial peptide sequence
TDRPYVL

SEQ ID NO: 317 - protein, 7 aa, Artificial Sequence
  Artificial peptide sequence
TDRPYVI

SEQ ID NO: 318 - protein, 7 aa, Artificial Sequence
  Artificial peptide sequence
TDRPYVV

SEQ ID NO: 319 - protein, 7 aa, Artificial Sequence
  Artificial peptide sequence
TDRPWIL

SEQ ID NO: 320 - protein, 7 aa, Artificial Sequence
  Artificial peptide sequence
TDRPWII

SEQ ID NO: 321 - protein, 7 aa, Artificial Sequence
  Artificial peptide sequence
TDRPWIV

SEQ ID NO: 322 - protein, 7 aa, Artificial Sequence
  Artificial peptide sequence
TDRPWLL

SEQ ID NO: 323 - protein, 7 aa, Artificial Sequence
  Artificial peptide sequence
TDRPWLI

SEQ ID NO: 324 - protein, 7 aa, Artificial Sequence
  Artificial peptide sequence
TDRPWLV

SEQ ID NO: 325 - protein, 7 aa, Artificial Sequence
  Artificial peptide sequence
TDRPWVL

SEQ ID NO: 326 - protein, 7 aa, Artificial Sequence
  Artificial peptide sequence
TDRPWVI

SEQ ID NO: 327 - protein, 7 aa, Artificial Sequence
  Artificial peptide sequence
TDRPWVV

SEQ ID NO: 328 - protein, 7 aa, Artificial Sequence
  Artificial peptide sequence
TEKPYIL

SEQ ID NO: 329 - protein, 7 aa, Artificial Sequence
  Artificial peptide sequence
TEKPYII

SEQ ID NO: 330 - protein, 7 aa, Artificial Sequence
  Artificial peptide sequence
TEKPYIV

SEQ ID NO: 331 - protein, 7 aa, Artificial Sequence
  Artificial peptide sequence
TEKPYLL

SEQ ID NO: 332 - protein, 7 aa, Artificial Sequence
  Artificial peptide sequence
TEKPYLI

SEQ ID NO: 333 - protein, 7 aa, Artificial Sequence
  Artificial peptide sequence
TEKPYLV

SEQ ID NO: 334 - protein, 7 aa, Artificial Sequence
  Artificial peptide sequence
TEKPYVL

SEQ ID NO: 335 - protein, 7 aa, Artificial Sequence
  Artificial peptide sequence
TEKPYVI

SEQ ID NO: 336 - protein, 7 aa, Artificial Sequence
  Artificial peptide sequence
TEKPYVV

SEQ ID NO: 337 - protein, 7 aa, Artificial Sequence
  Artificial peptide sequence
TEKPWIL

SEQ ID NO: 338 - protein, 7 aa, Artificial Sequence
  Artificial peptide sequence
TEKPWII

SEQ ID NO: 339 - protein, 7 aa, Artificial Sequence
  Artificial peptide sequence
TEKPWIV

SEQ ID NO: 340 - protein, 7 aa, Artificial Sequence
  Artificial peptide sequence
TEKPWLL

SEQ ID NO: 341 - protein, 7 aa, Artificial Sequence
  Artificial peptide sequence
TEKPWLI

SEQ ID NO: 342 - protein, 7 aa, Artificial Sequence
  Artificial peptide sequence
TEKPWLV

SEQ ID NO: 343 - protein, 7 aa, Artificial Sequence
  Artificial peptide sequence
TEKPWVL

SEQ ID NO: 344 - protein, 7 aa, Artificial Sequence
  Artificial peptide sequence
TEKPWVI

SEQ ID NO: 345 - protein, 7 aa, Artificial Sequence
  Artificial peptide sequence
TEKPWVV

SEQ ID NO: 346 - protein, 7 aa, Artificial Sequence
  Artificial peptide sequence
TERPYIL

SEQ ID NO: 347 - protein, 7 aa, Artificial Sequence
  Artificial peptide sequence
TERPYII

SEQ ID NO: 348 - protein, 7 aa, Artificial Sequence
  Artificial peptide sequence
TERPYIV

SEQ ID NO: 349 - protein, 7 aa, Artificial Sequence
  Artificial peptide sequence
TERPYLL

SEQ ID NO: 350 - protein, 7 aa, Artificial Sequence
  Artificial peptide sequence
TERPYLI

SEQ ID NO: 351 - protein, 7 aa, Artificial Sequence
  Artificial peptide sequence
TERPYLV

SEQ ID NO: 352 - protein, 7 aa, Artificial Sequence
  Artificial peptide sequence
TERPYVL

SEQ ID NO: 353 - protein, 7 aa, Artificial Sequence
  Artificial peptide sequence
TERPYVI

SEQ ID NO: 354 - protein, 7 aa, Artificial Sequence
  Artificial peptide sequence
TERPYVV

SEQ ID NO: 355 - protein, 7 aa, Artificial Sequence
  Artificial peptide sequence
TERPWIL

SEQ ID NO: 356 - protein, 7 aa, Artificial Sequence
  Artificial peptide sequence
TERPWII

SEQ ID NO: 357 - protein, 7 aa, Artificial Sequence
  Artificial peptide sequence
TERPWIV

SEQ ID NO: 358 - protein, 7 aa, Artificial Sequence
  Artificial peptide sequence
TERPWLL

SEQ ID NO: 359 - protein, 7 aa, Artificial Sequence
  Artificial peptide sequence
TERPWLI

SEQ ID NO: 360 - protein, 7 aa, Artificial Sequence
  Artificial peptide sequence
TERPWLV

SEQ ID NO: 361 - protein, 7 aa, Artificial Sequence
  Artificial peptide sequence
TERPWVL

SEQ ID NO: 362 - protein, 7 aa, Artificial Sequence
  Artificial peptide sequence
TERPWVI

SEQ ID NO: 363 - protein, 7 aa, Artificial Sequence
  Artificial peptide sequence
TERPWVV

SEQ ID NO: 364 - protein, 8 aa, Artificial Sequence
  Artificial peptide sequence
ASDKPYII

SEQ ID NO: 365 - protein, 8 aa, Artificial Sequence
  Artificial peptide sequence
ASDKPYIV

SEQ ID NO: 366 - protein, 8 aa, Artificial Sequence
  Artificial peptide sequence
ASDKPYLL

SEQ ID NO: 367 - protein, 8 aa, Artificial Sequence
  Artificial peptide sequence
ASDKPYLI

SEQ ID NO: 368 - protein, 8 aa, Artificial Sequence
  Artificial peptide sequence
ASDKPYLV

SEQ ID NO: 369 - protein, 8 aa, Artificial Sequence
  Artificial peptide sequence
ASDKPYVL

SEQ ID NO: 370 - protein, 8 aa, Artificial Sequence
  Artificial peptide sequence
ASDKPYVI

SEQ ID NO: 371 - protein, 8 aa, Artificial Sequence
  Artificial peptide sequence
ASDKPYVV

SEQ ID NO: 372 - protein, 8 aa, Artificial Sequence
  Artificial peptide sequence
ASDKPWIL

SEQ ID NO: 373 - protein, 8 aa, Artificial Sequence
  Artificial peptide sequence
ASDKPWII

SEQ ID NO: 374 - protein, 8 aa, Artificial Sequence
  Artificial peptide sequence
ASDKPWIV

SEQ ID NO: 375 - protein, 8 aa, Artificial Sequence
  Artificial peptide sequence
ASDKPWLL

SEQ ID NO: 376 - protein, 8 aa, Artificial Sequence
  Artificial peptide sequence
ASDKPWLI

SEQ ID NO: 377 - protein, 8 aa, Artificial Sequence
  Artificial peptide sequence
ASDKPWLV

SEQ ID NO: 378 - protein, 8 aa, Artificial Sequence
  Artificial peptide sequence
ASDKPWVL

SEQ ID NO: 379 - protein, 8 aa, Artificial Sequence
  Artificial peptide sequence
ASDKPWVI

SEQ ID NO: 380 - protein, 8 aa, Artificial Sequence
  Artificial peptide sequence
ASDKPWVV

SEQ ID NO: 381 - protein, 8 aa, Artificial Sequence
  Artificial peptide sequence
ASDRPYIL

SEQ ID NO: 382 - protein, 8 aa, Artificial Sequence
  Artificial peptide sequence
ASDRPYII

SEQ ID NO: 383 - protein, 8 aa, Artificial Sequence
  Artificial peptide sequence
ASDRPYIV

SEQ ID NO: 384 - protein, 8 aa, Artificial Sequence
  Artificial peptide sequence
ASDRPYLL

SEQ ID NO: 385 - protein, 8 aa, Artificial Sequence
  Artificial peptide sequence
ASDRPYLI

SEQ ID NO: 386 - protein, 8 aa, Artificial Sequence
  Artificial peptide sequence
ASDRPYLV

SEQ ID NO: 387 - protein, 8 aa, Artificial Sequence
  Artificial peptide sequence
ASDRPYVL

SEQ ID NO: 388 - protein, 8 aa, Artificial Sequence
  Artificial peptide sequence
ASDRPYVI

SEQ ID NO: 389 - protein, 8 aa, Artificial Sequence
  Artificial peptide sequence
ASDRPYVV

SEQ ID NO: 390 - protein, 8 aa, Artificial Sequence
  Artificial peptide sequence
ASDRPWIL

SEQ ID NO: 391 - protein, 8 aa, Artificial Sequence
  Artificial peptide sequence
ASDRPWII

SEQ ID NO: 392 - protein, 8 aa, Artificial Sequence
  Artificial peptide sequence
ASDRPWIV

SEQ ID NO: 393 - protein, 8 aa, Artificial Sequence
  Artificial peptide sequence
ASDRPWLL

SEQ ID NO: 394 - protein, 8 aa, Artificial Sequence
  Artificial peptide sequence
ASDRPWLI

SEQ ID NO: 395 - protein, 8 aa, Artificial Sequence
  Artificial peptide sequence
ASDRPWLV

SEQ ID NO: 396 - protein, 8 aa, Artificial Sequence
  Artificial peptide sequence
ASDRPWVL

SEQ ID NO: 397 - protein, 8 aa, Artificial Sequence
  Artificial peptide sequence
ASDRPWVI

SEQ ID NO: 398 - protein, 8 aa, Artificial Sequence
  Artificial peptide sequence
ASDRPWVV

SEQ ID NO: 399 - protein, 8 aa, Artificial Sequence
  Artificial peptide sequence
ASEKPYIL

SEQ ID NO: 400 - protein, 8 aa, Artificial Sequence
  Artificial peptide sequence
ASEKPYII

SEQ ID NO: 401 - protein, 8 aa, Artificial Sequence
  Artificial peptide sequence
ASEKPYIV

SEQ ID NO: 402 - protein, 8 aa, Artificial Sequence
  Artificial peptide sequence
ASEKPYLL

SEQ ID NO: 403 - protein, 8 aa, Artificial Sequence
  Artificial peptide sequence
ASEKPYLI

SEQ ID NO: 404 - protein, 8 aa, Artificial Sequence
  Artificial peptide sequence
ASEKPYLV

SEQ ID NO: 405 - protein, 8 aa, Artificial Sequence
  Artificial peptide sequence
ASEKPYVL

SEQ ID NO: 406 - protein, 8 aa, Artificial Sequence
  Artificial peptide sequence
ASEKPYVI

SEQ ID NO: 407 - protein, 8 aa, Artificial Sequence
  Artificial peptide sequence
ASEKPYVV

SEQ ID NO: 408 - protein, 8 aa, Artificial Sequence
  Artificial peptide sequence
ASEKPWIL

SEQ ID NO: 409 - protein, 8 aa, Artificial Sequence
  Artificial peptide sequence
ASEKPWII

SEQ ID NO: 410 - protein, 8 aa, Artificial Sequence
  Artificial peptide sequence
ASEKPWIV

SEQ ID NO: 411 - protein, 8 aa, Artificial Sequence
  Artificial peptide sequence
ASEKPWLL

SEQ ID NO: 412 - protein, 8 aa, Artificial Sequence
  Artificial peptide sequence
ASEKPWLI

SEQ ID NO: 413 - protein, 8 aa, Artificial Sequence
  Artificial peptide sequence
ASEKPWLV

SEQ ID NO: 414 - protein, 8 aa, Artificial Sequence
  Artificial peptide sequence
ASEKPWVL

SEQ ID NO: 415 - protein, 8 aa, Artificial Sequence
  Artificial peptide sequence
ASEKPWVI

SEQ ID NO: 416 - protein, 8 aa, Artificial Sequence
  Artificial peptide sequence
ASEKPWVV

SEQ ID NO: 417 - protein, 8 aa, Artificial Sequence
  Artificial peptide sequence
ASERPYIL

SEQ ID NO: 418 - protein, 8 aa, Artificial Sequence
  Artificial peptide sequence
ASERPYII

SEQ ID NO: 419 - protein, 8 aa, Artificial Sequence
  Artificial peptide sequence
ASERPYIV

SEQ ID NO: 420 - protein, 8 aa, Artificial Sequence
  Artificial peptide sequence
ASERPYLL

SEQ ID NO: 421 - protein, 8 aa, Artificial Sequence
  Artificial peptide sequence
ASERPYLI

SEQ ID NO: 422 - protein, 8 aa, Artificial Sequence
  Artificial peptide sequence
ASERPYLV

SEQ ID NO: 423 - protein, 8 aa, Artificial Sequence
  Artificial peptide sequence
ASERPYVL

SEQ ID NO: 424 - protein, 8 aa, Artificial Sequence
  Artificial peptide sequence
ASERPYVI

SEQ ID NO: 425 - protein, 8 aa, Artificial Sequence
  Artificial peptide sequence
ASERPYVV

SEQ ID NO: 426 - protein, 8 aa, Artificial Sequence
  Artificial peptide sequence
ASERPWIL

SEQ ID NO: 427 - protein, 8 aa, Artificial Sequence
  Artificial peptide sequence
ASERPWII

SEQ ID NO: 428 - protein, 8 aa, Artificial Sequence
  Artificial peptide sequence
ASERPWIV

SEQ ID NO: 429 - protein, 8 aa, Artificial Sequence
  Artificial peptide sequence
ASERPWLL

SEQ ID NO: 430 - protein, 8 aa, Artificial Sequence
  Artificial peptide sequence
ASERPWLI

SEQ ID NO: 431 - protein, 8 aa, Artificial Sequence
  Artificial peptide sequence
ASERPWLV

SEQ ID NO: 432 - protein, 8 aa, Artificial Sequence
  Artificial peptide sequence
ASERPWVL

SEQ ID NO: 433 - protein, 8 aa, Artificial Sequence
  Artificial peptide sequence
ASERPWVI

SEQ ID NO: 434 - protein, 8 aa, Artificial Sequence
  Artificial peptide sequence
ASERPWVV

SEQ ID NO: 435 - protein, 8 aa, Artificial Sequence
  Artificial peptide sequence
ATDKPYIL

SEQ ID NO: 436 - protein, 8 aa, Artificial Sequence
  Artificial peptide sequence
ATDKPYII

SEQ ID NO: 437 - protein, 8 aa, Artificial Sequence
  Artificial peptide sequence
ATDKPYIV

SEQ ID NO: 438 - protein, 8 aa, Artificial Sequence
  Artificial peptide sequence
ATDKPYLL

SEQ ID NO: 439 - protein, 8 aa, Artificial Sequence
  Artificial peptide sequence
ATDKPYLI

SEQ ID NO: 440 - protein, 8 aa, Artificial Sequence
  Artificial peptide sequence
ATDKPYLV

SEQ ID NO: 441 - protein, 8 aa, Artificial Sequence
  Artificial peptide sequence
ATDKPYVL

SEQ ID NO: 442 - protein, 8 aa, Artificial Sequence
  Artificial peptide sequence
ATDKPYVI

SEQ ID NO: 443 - protein, 8 aa, Artificial Sequence
  Artificial peptide sequence
ATDKPYVV

SEQ ID NO: 444 - protein, 8 aa, Artificial Sequence
  Artificial peptide sequence
ATDKPWIL

SEQ ID NO: 445 - protein, 8 aa, Artificial Sequence
  Artificial peptide sequence
ATDKPWII

SEQ ID NO: 446 - protein, 8 aa, Artificial Sequence
  Artificial peptide sequence
ATDKPWIV

SEQ ID NO: 447 - protein, 8 aa, Artificial Sequence
  Artificial peptide sequence
ATDKPWLL

SEQ ID NO: 448 - protein, 8 aa, Artificial Sequence
  Artificial peptide sequence
ATDKPWLI

SEQ ID NO: 449 - protein, 8 aa, Artificial Sequence
  Artificial peptide sequence
ATDKPWLV

SEQ ID NO: 450 - protein, 8 aa, Artificial Sequence
  Artificial peptide sequence
ATDKPWVL

SEQ ID NO: 451 - protein, 8 aa, Artificial Sequence
  Artificial peptide sequence
ATDKPWVI

SEQ ID NO: 452 - protein, 8 aa, Artificial Sequence
  Artificial peptide sequence
ATDKPWVV

SEQ ID NO: 453 - protein, 8 aa, Artificial Sequence
  Artificial peptide sequence
ATDRPYIL

SEQ ID NO: 454 - protein, 8 aa, Artificial Sequence
  Artificial peptide sequence
ATDRPYII

SEQ ID NO: 455 - protein, 8 aa, Artificial Sequence
  Artificial peptide sequence
ATDRPYIV

SEQ ID NO: 456 - protein, 8 aa, Artificial Sequence
  Artificial peptide sequence
ATDRPYLL

SEQ ID NO: 457 - protein, 8 aa, Artificial Sequence
  Artificial peptide sequence
ATDRPYLI

SEQ ID NO: 458 - protein, 8 aa, Artificial Sequence
  Artificial peptide sequence
ATDRPYLV

SEQ ID NO: 459 - protein, 8 aa, Artificial Sequence
  Artificial peptide sequence
ATDRPYVL

SEQ ID NO: 460 - protein, 8 aa, Artificial Sequence
  Artificial peptide sequence
ATDRPYVI

SEQ ID NO: 461 - protein, 8 aa, Artificial Sequence
  Artificial peptide sequence
ATDRPYVV

SEQ ID NO: 462 - protein, 8 aa, Artificial Sequence
  Artificial peptide sequence
ATDRPWIL

SEQ ID NO: 463 - protein, 8 aa, Artificial Sequence
  Artificial peptide sequence
ATDRPWII

SEQ ID NO: 464 - protein, 8 aa, Artificial Sequence
  Artificial peptide sequence
ATDRPWIV

SEQ ID NO: 465 - protein, 8 aa, Artificial Sequence
  Artificial peptide sequence
ATDRPWLL

SEQ ID NO: 466 - protein, 8 aa, Artificial Sequence
  Artificial peptide sequence
ATDRPWLI

SEQ ID NO: 467 - protein, 8 aa, Artificial Sequence
  Artificial peptide sequence
ATDRPWLV

SEQ ID NO: 468 - protein, 8 aa, Artificial Sequence
  Artificial peptide sequence
ATDRPWVL

SEQ ID NO: 469 - protein, 8 aa, Artificial Sequence
  Artificial peptide sequence
ATDRPWVI

SEQ ID NO: 470 - protein, 8 aa, Artificial Sequence
  Artificial peptide sequence
ATDRPWVV

SEQ ID NO: 471 - protein, 8 aa, Artificial Sequence
  Artificial peptide sequence
ATEKPYIL

SEQ ID NO: 472 - protein, 8 aa, Artificial Sequence
  Artificial peptide sequence
ATEKPYII

SEQ ID NO: 473 - protein, 8 aa, Artificial Sequence
  Artificial peptide sequence
ATEKPYIV

SEQ ID NO: 474 - protein, 8 aa, Artificial Sequence
  Artificial peptide sequence
ATEKPYLL

SEQ ID NO: 475 - protein, 8 aa, Artificial Sequence
  Artificial peptide sequence
ATEKPYLI

SEQ ID NO: 476 - protein, 8 aa, Artificial Sequence
  Artificial peptide sequence
ATEKPYLV

SEQ ID NO: 477 - protein, 8 aa, Artificial Sequence
  Artificial peptide sequence
ATEKPYVL

SEQ ID NO: 478 - protein, 8 aa, Artificial Sequence
  Artificial peptide sequence
ATEKPYVI

SEQ ID NO: 479 - protein, 8 aa, Artificial Sequence
  Artificial peptide sequence
ATEKPYVV

SEQ ID NO: 480 - protein, 8 aa, Artificial Sequence
  Artificial peptide sequence
ATEKPWIL

SEQ ID NO: 481 - protein, 8 aa, Artificial Sequence
  Artificial peptide sequence
ATEKPWII

SEQ ID NO: 482 - protein, 8 aa, Artificial Sequence
  Artificial peptide sequence
ATEKPWIV

SEQ ID NO: 483 - protein, 8 aa, Artificial Sequence
  Artificial peptide sequence
ATEKPWLL

SEQ ID NO: 484 - protein, 8 aa, Artificial Sequence
  Artificial peptide sequence
ATEKPWLI

SEQ ID NO: 485 - protein, 8 aa, Artificial Sequence
  Artificial peptide sequence
ATEKPWLV

SEQ ID NO: 486 - protein, 8 aa, Artificial Sequence
  Artificial peptide sequence
ATEKPWVL

SEQ ID NO: 487 - protein, 8 aa, Artificial Sequence
  Artificial peptide sequence
ATEKPWVI

SEQ ID NO: 488 - protein, 8 aa, Artificial Sequence
  Artificial peptide sequence
ATEKPWVV

SEQ ID NO: 489 - protein, 8 aa, Artificial Sequence
  Artificial peptide sequence
ATERPYIL

SEQ ID NO: 490 - protein, 8 aa, Artificial Sequence
  Artificial peptide sequence
ATERPYII

SEQ ID NO: 491 - protein, 8 aa, Artificial Sequence
  Artificial peptide sequence
ATERPYIV

SEQ ID NO: 492 - protein, 8 aa, Artificial Sequence
  Artificial peptide sequence
ATERPYLL

SEQ ID NO: 493 - protein, 8 aa, Artificial Sequence
  Artificial peptide sequence
ATERPYLI

SEQ ID NO: 494 - protein, 8 aa, Artificial Sequence
  Artificial peptide sequence
ATERPYLV

SEQ ID NO: 495 - protein, 8 aa, Artificial Sequence
  Artificial peptide sequence
ATERPYVL

SEQ ID NO: 496 - protein, 8 aa, Artificial Sequence
  Artificial peptide sequence
ATERPYVI

SEQ ID NO: 497 - protein, 8 aa, Artificial Sequence
  Artificial peptide sequence
ATERPYVV

SEQ ID NO: 498 - protein, 8 aa, Artificial Sequence
  Artificial peptide sequence
ATERPWIL

SEQ ID NO: 499 - protein, 8 aa, Artificial Sequence
  Artificial peptide sequence
ATERPWII

SEQ ID NO: 500 - protein, 8 aa, Artificial Sequence
  Artificial peptide sequence
ATERPWIV

SEQ ID NO: 501 - protein, 8 aa, Artificial Sequence
  Artificial peptide sequence
ATERPWLL

SEQ ID NO: 502 - protein, 8 aa, Artificial Sequence
  Artificial peptide sequence
ATERPWLI

SEQ ID NO: 503 - protein, 8 aa, Artificial Sequence
  Artificial peptide sequence
ATERPWLV

SEQ ID NO: 504 - protein, 8 aa, Artificial Sequence
  Artificial peptide sequence
ATERPWVL

SEQ ID NO: 505 - protein, 8 aa, Artificial Sequence
  Artificial peptide sequence
ATERPWVI

SEQ ID NO: 506 - protein, 8 aa, Artificial Sequence
  Artificial peptide sequence
ATERPWVV

SEQ ID NO: 507 - protein, 8 aa, Artificial Sequence
  Artificial peptide sequence
LSDKPYIL

SEQ ID NO: 508 - protein, 8 aa, Artificial Sequence
  Artificial peptide sequence
LSDKPYII

SEQ ID NO: 509 - protein, 8 aa, Artificial Sequence
  Artificial peptide sequence
LSDKPYIV

SEQ ID NO: 510 - protein, 8 aa, Artificial Sequence
  Artificial peptide sequence
LSDKPYLL

SEQ ID NO: 511 - protein, 8 aa, Artificial Sequence
  Artificial peptide sequence
LSDKPYLI

SEQ ID NO: 512 - protein, 8 aa, Artificial Sequence
  Artificial peptide sequence
LSDKPYLV

SEQ ID NO: 513 - protein, 8 aa, Artificial Sequence
  Artificial peptide sequence
LSDKPYVL

SEQ ID NO: 514 - protein, 8 aa, Artificial Sequence
  Artificial peptide sequence
LSDKPYVI

SEQ ID NO: 515 - protein, 8 aa, Artificial Sequence
  Artificial peptide sequence
LSDKPYVV

SEQ ID NO: 516 - protein, 8 aa, Artificial Sequence
  Artificial peptide sequence
LSDKPWIL

SEQ ID NO: 517 - protein, 8 aa, Artificial Sequence
  Artificial peptide sequence
LSDKPWII

SEQ ID NO: 518 - protein, 8 aa, Artificial Sequence
  Artificial peptide sequence
LSDKPWIV

SEQ ID NO: 519 - protein, 8 aa, Artificial Sequence
  Artificial peptide sequence
LSDKPWLL

SEQ ID NO: 520 - protein, 8 aa, Artificial Sequence
  Artificial peptide sequence
LSDKPWLI

SEQ ID NO: 521 - protein, 8 aa, Artificial Sequence
  Artificial peptide sequence
LSDKPWLV

SEQ ID NO: 522 - protein, 8 aa, Artificial Sequence
  Artificial peptide sequence
LSDKPWVL

SEQ ID NO: 523 - protein, 8 aa, Artificial Sequence
  Artificial peptide sequence
LSDKPWVI

SEQ ID NO: 524 - protein, 8 aa, Artificial Sequence
  Artificial peptide sequence
LSDKPWVV

SEQ ID NO: 525 - protein, 8 aa, Artificial Sequence
  Artificial peptide sequence
LSDRPYIL

SEQ ID NO: 526 - protein, 8 aa, Artificial Sequence
  Artificial peptide sequence
LSDRPYII

SEQ ID NO: 527 - protein, 8 aa, Artificial Sequence
  Artificial peptide sequence
LSDRPYIV

SEQ ID NO: 528 - protein, 8 aa, Artificial Sequence
  Artificial peptide sequence
LSDRPYLL

SEQ ID NO: 529 - protein, 8 aa, Artificial Sequence
  Artificial peptide sequence
LSDRPYLI

SEQ ID NO: 530 - protein, 8 aa, Artificial Sequence
  Artificial peptide sequence
LSDRPYLV

SEQ ID NO: 531 - protein, 8 aa, Artificial Sequence
  Artificial peptide sequence
LSDRPYVL

SEQ ID NO: 532 - protein, 8 aa, Artificial Sequence
  Artificial peptide sequence
LSDRPYVI

SEQ ID NO: 533 - protein, 8 aa, Artificial Sequence
  Artificial peptide sequence
LSDRPYVV

SEQ ID NO: 534 - protein, 8 aa, Artificial Sequence
  Artificial peptide sequence
LSDRPWIL

SEQ ID NO: 535 - protein, 8 aa, Artificial Sequence
  Artificial peptide sequence
LSDRPWII

SEQ ID NO: 536 - protein, 8 aa, Artificial Sequence
  Artificial peptide sequence
LSDRPWIV

SEQ ID NO: 537 - protein, 8 aa, Artificial Sequence
  Artificial peptide sequence
LSDRPWLL

SEQ ID NO: 538 - protein, 8 aa, Artificial Sequence
  Artificial peptide sequence
LSDRPWLI

SEQ ID NO: 539 - protein, 8 aa, Artificial Sequence
  Artificial peptide sequence
LSDRPWLV

SEQ ID NO: 540 - protein, 8 aa, Artificial Sequence
  Artificial peptide sequence
LSDRPWVL

SEQ ID NO: 541 - protein, 8 aa, Artificial Sequence
  Artificial peptide sequence
LSDRPWVI

SEQ ID NO: 542 - protein, 8 aa, Artificial Sequence
  Artificial peptide sequence
LSDRPWVV

SEQ ID NO: 543 - protein, 8 aa, Artificial Sequence
  Artificial peptide sequence
LSEKPYIL

SEQ ID NO: 544 - protein, 8 aa, Artificial Sequence
  Artificial peptide sequence
LSEKPYII

SEQ ID NO: 545 - protein, 8 aa, Artificial Sequence
  Artificial peptide sequence
LSEKPYIV

SEQ ID NO: 546 - protein, 8 aa, Artificial Sequence
  Artificial peptide sequence
LSEKPYLL

SEQ ID NO: 547 - protein, 8 aa, Artificial Sequence
  Artificial peptide sequence
LSEKPYLI

SEQ ID NO: 548 - protein, 8 aa, Artificial Sequence
  Artificial peptide sequence
LSEKPYLV

SEQ ID NO: 549 - protein, 8 aa, Artificial Sequence
  Artificial peptide sequence
LSEKPYVL

SEQ ID NO: 550 - protein, 8 aa, Artificial Sequence
  Artificial peptide sequence
LSEKPYVI

SEQ ID NO: 551 - protein, 8 aa, Artificial Sequence
  Artificial peptide sequence
LSEKPYVV

SEQ ID NO: 552 - protein, 8 aa, Artificial Sequence
  Artificial peptide sequence
LSEKPWIL

SEQ ID NO: 553 - protein, 8 aa, Artificial Sequence
  Artificial peptide sequence
LSEKPWII

SEQ ID NO: 554 - protein, 8 aa, Artificial Sequence
  Artificial peptide sequence
LSEKPWIV

SEQ ID NO: 555 - protein, 8 aa, Artificial Sequence
  Artificial peptide sequence
LSEKPWLL

SEQ ID NO: 556 - protein, 8 aa, Artificial Sequence
  Artificial peptide sequence
LSEKPWLI

SEQ ID NO: 557 - protein, 8 aa, Artificial Sequence
  Artificial peptide sequence
LSEKPWLV

SEQ ID NO: 558 - protein, 8 aa, Artificial Sequence
  Artificial peptide sequence
LSEKPWVL

SEQ ID NO: 559 - protein, 8 aa, Artificial Sequence
  Artificial peptide sequence
LSEKPWVI

SEQ ID NO: 560 - protein, 8 aa, Artificial Sequence
  Artificial peptide sequence
LSEKPWVV

SEQ ID NO: 561 - protein, 8 aa, Artificial Sequence
  Artificial peptide sequence
LSERPYIL

SEQ ID NO: 562 - protein, 8 aa, Artificial Sequence
  Artificial peptide sequence
LSERPYII

SEQ ID NO: 563 - protein, 8 aa, Artificial Sequence
  Artificial peptide sequence
LSERPYIV

SEQ ID NO: 564 - protein, 8 aa, Artificial Sequence
  Artificial peptide sequence
LSERPYLL

SEQ ID NO: 565 - protein, 8 aa, Artificial Sequence
  Artificial peptide sequence
LSERPYLI

SEQ ID NO: 566 - protein, 8 aa, Artificial Sequence
  Artificial peptide sequence
LSERPYLV

SEQ ID NO: 567 - protein, 8 aa, Artificial Sequence
  Artificial peptide sequence
LSERPYVL

SEQ ID NO: 568 - protein, 8 aa, Artificial Sequence
  Artificial peptide sequence
LSERPYVI

SEQ ID NO: 569 - protein, 8 aa, Artificial Sequence
  Artificial peptide sequence
LSERPYVV

SEQ ID NO: 570 - protein, 8 aa, Artificial Sequence
  Artificial peptide sequence
LSERPWIL

SEQ ID NO: 571 - protein, 8 aa, Artificial Sequence
  Artificial peptide sequence
LSERPWII

SEQ ID NO: 572 - protein, 8 aa, Artificial Sequence
  Artificial peptide sequence
LSERPWIV

SEQ ID NO: 573 - protein, 8 aa, Artificial Sequence
  Artificial peptide sequence
LSERPWLL

SEQ ID NO: 574 - protein, 8 aa, Artificial Sequence
  Artificial peptide sequence
LSERPWLI

SEQ ID NO: 575 - protein, 8 aa, Artificial Sequence
  Artificial peptide sequence
LSERPWLV

SEQ ID NO: 576 - protein, 8 aa, Artificial Sequence
  Artificial peptide sequence
LSERPWVL

SEQ ID NO: 577 - protein, 8 aa, Artificial Sequence
  Artificial peptide sequence
LSERPWVI

SEQ ID NO: 578 - protein, 8 aa, Artificial Sequence
  Artificial peptide sequence
LSERPWVV

SEQ ID NO: 579 - protein, 8 aa, Artificial Sequence
  Artificial peptide sequence
LTDKPYIL

SEQ ID NO: 580 - protein, 8 aa, Artificial Sequence
  Artificial peptide sequence
LTDKPYII

SEQ ID NO: 581 - protein, 8 aa, Artificial Sequence
  Artificial peptide sequence
LTDKPYIV

SEQ ID NO: 582 - protein, 8 aa, Artificial Sequence
  Artificial peptide sequence
LTDKPYLL

SEQ ID NO: 583 - protein, 8 aa, Artificial Sequence
  Artificial peptide sequence
LTDKPYLI

SEQ ID NO: 584 - protein, 8 aa, Artificial Sequence
  Artificial peptide sequence
LTDKPYLV

SEQ ID NO: 585 - protein, 8 aa, Artificial Sequence
  Artificial peptide sequence
LTDKPYVL

SEQ ID NO: 586 - protein, 8 aa, Artificial Sequence
  Artificial peptide sequence
LTDKPYVI

SEQ ID NO: 587 - protein, 8 aa, Artificial Sequence
  Artificial peptide sequence
LTDKPYVV

SEQ ID NO: 588 - protein, 8 aa, Artificial Sequence
  Artificial peptide sequence
LTDKPWIL

SEQ ID NO: 589 - protein, 8 aa, Artificial Sequence
  Artificial peptide sequence
LTDKPWII

SEQ ID NO: 590 - protein, 8 aa, Artificial Sequence
  Artificial peptide sequence
LTDKPWIV

SEQ ID NO: 591 - protein, 8 aa, Artificial Sequence
  Artificial peptide sequence
LTDKPWLL

SEQ ID NO: 592 - protein, 8 aa, Artificial Sequence
  Artificial peptide sequence
LTDKPWLI

SEQ ID NO: 593 - protein, 8 aa, Artificial Sequence
  Artificial peptide sequence
LTDKPWLV

SEQ ID NO: 594 - protein, 8 aa, Artificial Sequence
  Artificial peptide sequence
LTDKPWVL

SEQ ID NO: 595 - protein, 8 aa, Artificial Sequence
  Artificial peptide sequence
LTDKPWVI

SEQ ID NO: 596 - protein, 8 aa, Artificial Sequence
  Artificial peptide sequence
LTDKPWVV

SEQ ID NO: 597 - protein, 8 aa, Artificial Sequence
  Artificial peptide sequence
LTDRPYIL

SEQ ID NO: 598 - protein, 8 aa, Artificial Sequence
  Artificial peptide sequence
LTDRPYII

SEQ ID NO: 599 - protein, 8 aa, Artificial Sequence
  Artificial peptide sequence
LTDRPYIV

SEQ ID NO: 600 - protein, 8 aa, Artificial Sequence
  Artificial peptide sequence
LTDRPYLL

SEQ ID NO: 601 - protein, 8 aa, Artificial Sequence
  Artificial peptide sequence
LTDRPYLI

SEQ ID NO: 602 - protein, 8 aa, Artificial Sequence
  Artificial peptide sequence
LTDRPYLV

SEQ ID NO: 603 - protein, 8 aa, Artificial Sequence
  Artificial peptide sequence
LTDRPYVL

SEQ ID NO: 604 - protein, 8 aa, Artificial Sequence
  Artificial peptide sequence
LTDRPYVI

SEQ ID NO: 605 - protein, 8 aa, Artificial Sequence
  Artificial peptide sequence
LTDRPYVV

SEQ ID NO: 606 - protein, 8 aa, Artificial Sequence
  Artificial peptide sequence
LTDRPWIL

SEQ ID NO: 607 - protein, 8 aa, Artificial Sequence
  Artificial peptide sequence
LTDRPWII

SEQ ID NO: 608 - protein, 8 aa, Artificial Sequence
  Artificial peptide sequence
LTDRPWIV

SEQ ID NO: 609 - protein, 8 aa, Artificial Sequence
  Artificial peptide sequence
LTDRPWLL

SEQ ID NO: 610 - protein, 8 aa, Artificial Sequence
  Artificial peptide sequence
LTDRPWLI

SEQ ID NO: 611 - protein, 8 aa, Artificial Sequence
  Artificial peptide sequence
LTDRPWLV

SEQ ID NO: 612 - protein, 8 aa, Artificial Sequence
  Artificial peptide sequence
LTDRPWVL

SEQ ID NO: 613 - protein, 8 aa, Artificial Sequence
  Artificial peptide sequence
LTDRPWVI

SEQ ID NO: 614 - protein, 8 aa, Artificial Sequence
  Artificial peptide sequence
LTDRPWVV

SEQ ID NO: 615 - protein, 8 aa, Artificial Sequence
  Artificial peptide sequence
LTEKPYIL

SEQ ID NO: 616 - protein, 8 aa, Artificial Sequence
  Artificial peptide sequence
LTEKPYII

SEQ ID NO: 617 - protein, 8 aa, Artificial Sequence
  Artificial peptide sequence
LTEKPYIV

SEQ ID NO: 618 - protein, 8 aa, Artificial Sequence
  Artificial peptide sequence
LTEKPYLL

SEQ ID NO: 619 - protein, 8 aa, Artificial Sequence
  Artificial peptide sequence
LTEKPYLI

SEQ ID NO: 620 - protein, 8 aa, Artificial Sequence
  Artificial peptide sequence
LTEKPYLV

SEQ ID NO: 621 - protein, 8 aa, Artificial Sequence
  Artificial peptide sequence
LTEKPYVL

SEQ ID NO: 622 - protein, 8 aa, Artificial Sequence
  Artificial peptide sequence
LTEKPYVI

SEQ ID NO: 623 - protein, 8 aa, Artificial Sequence
  Artificial peptide sequence
LTEKPYVV

SEQ ID NO: 624 - protein, 8 aa, Artificial Sequence
  Artificial peptide sequence
LTEKPWIL

SEQ ID NO: 625 - protein, 8 aa, Artificial Sequence
  Artificial peptide sequence
LTEKPWII

SEQ ID NO: 626 - protein, 8 aa, Artificial Sequence
  Artificial peptide sequence
LTEKPWIV

SEQ ID NO: 627 - protein, 8 aa, Artificial Sequence
  Artificial peptide sequence
LTEKPWLL

SEQ ID NO: 628 - protein, 8 aa, Artificial Sequence
  Artificial peptide sequence
LTEKPWLI

SEQ ID NO: 629 - protein, 8 aa, Artificial Sequence
  Artificial peptide sequence
LTEKPWLV

SEQ ID NO: 630 - protein, 8 aa, Artificial Sequence
  Artificial peptide sequence
LTEKPWVL

SEQ ID NO: 631 - protein, 8 aa, Artificial Sequence
  Artificial peptide sequence
LTEKPWVI

SEQ ID NO: 632 - protein, 8 aa, Artificial Sequence
  Artificial peptide sequence
LTEKPWVV

SEQ ID NO: 633 - protein, 8 aa, Artificial Sequence
  Artificial peptide sequence
LTERPYIL

SEQ ID NO: 634 - protein, 8 aa, Artificial Sequence
  Artificial peptide sequence
LTERPYII

SEQ ID NO: 635 - protein, 8 aa, Artificial Sequence
  Artificial peptide sequence
LTERPYIV

SEQ ID NO: 636 - protein, 8 aa, Artificial Sequence
  Artificial peptide sequence
LTERPYLL

SEQ ID NO: 637 - protein, 8 aa, Artificial Sequence
  Artificial peptide sequence
LTERPYLI

SEQ ID NO: 638 - protein, 8 aa, Artificial Sequence
  Artificial peptide sequence
LTERPYLV

SEQ ID NO: 639 - protein, 8 aa, Artificial Sequence
  Artificial peptide sequence
LTERPYVL

SEQ ID NO: 640 - protein, 8 aa, Artificial Sequence
  Artificial peptide sequence
LTERPYVI

SEQ ID NO: 641 - protein, 8 aa, Artificial Sequence
  Artificial peptide sequence
LTERPYVV

SEQ ID NO: 642 - protein, 8 aa, Artificial Sequence
  Artificial peptide sequence
LTERPWIL

SEQ ID NO: 643 - protein, 8 aa, Artificial Sequence
  Artificial peptide sequence
LTERPWII

SEQ ID NO: 644 - protein, 8 aa, Artificial Sequence
  Artificial peptide sequence
LTERPWIV

SEQ ID NO: 645 - protein, 8 aa, Artificial Sequence
  Artificial peptide sequence
LTERPWLL

SEQ ID NO: 646 - protein, 8 aa, Artificial Sequence
  Artificial peptide sequence
LTERPWLI

SEQ ID NO: 647 - protein, 8 aa, Artificial Sequence
  Artificial peptide sequence
LTERPWLV

SEQ ID NO: 648 - protein, 8 aa, Artificial Sequence
  Artificial peptide sequence
LTERPWVL

SEQ ID NO: 649 - protein, 8 aa, Artificial Sequence
  Artificial peptide sequence
LTERPWVI

SEQ ID NO: 650 - protein, 8 aa, Artificial Sequence
  Artificial peptide sequence
LTERPWVV

SEQ ID NO: 651 - protein, 8 aa, Artificial Sequence
  Artificial peptide sequence
ISDKPYIL

SEQ ID NO: 652 - protein, 8 aa, Artificial Sequence
  Artificial peptide sequence
ISDKPYII

SEQ ID NO: 653 - protein, 8 aa, Artificial Sequence
  Artificial peptide sequence
ISDKPYIV

SEQ ID NO: 654 - protein, 8 aa, Artificial Sequence
  Artificial peptide sequence
ISDKPYLL

SEQ ID NO: 655 - protein, 8 aa, Artificial Sequence
  Artificial peptide sequence
ISDKPYLI

SEQ ID NO: 656 - protein, 8 aa, Artificial Sequence
  Artificial peptide sequence
ISDKPYLV

SEQ ID NO: 657 - protein, 8 aa, Artificial Sequence
  Artificial peptide sequence
ISDKPYVL

SEQ ID NO: 658 - protein, 8 aa, Artificial Sequence
  Artificial peptide sequence
ISDKPYVI

SEQ ID NO: 659 - protein, 8 aa, Artificial Sequence
  Artificial peptide sequence
ISDKPYVV

SEQ ID NO: 660 - protein, 8 aa, Artificial Sequence
  Artificial peptide sequence
ISDKPWIL

SEQ ID NO: 661 - protein, 8 aa, Artificial Sequence
  Artificial peptide sequence
ISDKPWII

SEQ ID NO: 662 - protein, 8 aa, Artificial Sequence
  Artificial peptide sequence
ISDKPWIV

SEQ ID NO: 663 - protein, 8 aa, Artificial Sequence
  Artificial peptide sequence
ISDKPWLL

SEQ ID NO: 664 - protein, 8 aa, Artificial Sequence
  Artificial peptide sequence
ISDKPWLI

SEQ ID NO: 665 - protein, 8 aa, Artificial Sequence
  Artificial peptide sequence
ISDKPWLV

SEQ ID NO: 666 - protein, 8 aa, Artificial Sequence
  Artificial peptide sequence
ISDKPWVL

SEQ ID NO: 667 - protein, 8 aa, Artificial Sequence
  Artificial peptide sequence
ISDKPWVI

SEQ ID NO: 668 - protein, 8 aa, Artificial Sequence
  Artificial peptide sequence
ISDKPWVV

SEQ ID NO: 669 - protein, 8 aa, Artificial Sequence
  Artificial peptide sequence
ISDRPYIL

SEQ ID NO: 670 - protein, 8 aa, Artificial Sequence
  Artificial peptide sequence
ISDRPYII

SEQ ID NO: 671 - protein, 8 aa, Artificial Sequence
  Artificial peptide sequence
ISDRPYIV

SEQ ID NO: 672 - protein, 8 aa, Artificial Sequence
  Artificial peptide sequence
ISDRPYLL

SEQ ID NO: 673 - protein, 8 aa, Artificial Sequence
  Artificial peptide sequence
ISDRPYLI

SEQ ID NO: 674 - protein, 8 aa, Artificial Sequence
  Artificial peptide sequence
ISDRPYLV

SEQ ID NO: 675 - protein, 8 aa, Artificial Sequence
  Artificial peptide sequence
ISDRPYVL

SEQ ID NO: 676 - protein, 8 aa, Artificial Sequence
  Artificial peptide sequence
ISDRPYVI

SEQ ID NO: 677 - protein, 8 aa, Artificial Sequence
  Artificial peptide sequence
ISDRPYVV

SEQ ID NO: 678 - protein, 8 aa, Artificial Sequence
  Artificial peptide sequence
ISDRPWIL

SEQ ID NO: 679 - protein, 8 aa, Artificial Sequence
  Artificial peptide sequence
ISDRPWII

SEQ ID NO: 680 - protein, 8 aa, Artificial Sequence
  Artificial peptide sequence
ISDRPWIV

SEQ ID NO: 681 - protein, 8 aa, Artificial Sequence
  Artificial peptide sequence
ISDRPWLL

SEQ ID NO: 682 - protein, 8 aa, Artificial Sequence
  Artificial peptide sequence
ISDRPWLI

SEQ ID NO: 683 - protein, 8 aa, Artificial Sequence
  Artificial peptide sequence
ISDRPWLV

SEQ ID NO: 684 - protein, 8 aa, Artificial Sequence
  Artificial peptide sequence
ISDRPWVL

SEQ ID NO: 685 - protein, 8 aa, Artificial Sequence
  Artificial peptide sequence
ISDRPWVI

SEQ ID NO: 686 - protein, 8 aa, Artificial Sequence
  Artificial peptide sequence
ISDRPWVV

SEQ ID NO: 687 - protein, 8 aa, Artificial Sequence
  Artificial peptide sequence
ISEKPYIL

SEQ ID NO: 688 - protein, 8 aa, Artificial Sequence
  Artificial peptide sequence
ISEKPYII

SEQ ID NO: 689 - protein, 8 aa, Artificial Sequence
  Artificial peptide sequence
ISEKPYIV

SEQ ID NO: 690 - protein, 8 aa, Artificial Sequence
  Artificial peptide sequence
ISEKPYLL

SEQ ID NO: 691 - protein, 8 aa, Artificial Sequence
  Artificial peptide sequence
ISEKPYLI

SEQ ID NO: 692 - protein, 8 aa, Artificial Sequence
  Artificial peptide sequence
ISEKPYLV

SEQ ID NO: 693 - protein, 8 aa, Artificial Sequence
  Artificial peptide sequence
ISEKPYVL

SEQ ID NO: 694 - protein, 8 aa, Artificial Sequence
  Artificial peptide sequence
ISEKPYVI

SEQ ID NO: 695 - protein, 8 aa, Artificial Sequence
  Artificial peptide sequence
ISEKPYVV

SEQ ID NO: 696 - protein, 8 aa, Artificial Sequence
  Artificial peptide sequence
ISEKPWIL

SEQ ID NO: 697 - protein, 8 aa, Artificial Sequence
  Artificial peptide sequence
ISEKPWII

SEQ ID NO: 698 - protein, 8 aa, Artificial Sequence
  Artificial peptide sequence
ISEKPWIV

SEQ ID NO: 699 - protein, 8 aa, Artificial Sequence
  Artificial peptide sequence
ISEKPWLL

SEQ ID NO: 700 - protein, 8 aa, Artificial Sequence
  Artificial peptide sequence
ISEKPWLI

SEQ ID NO: 701 - protein, 8 aa, Artificial Sequence
  Artificial peptide sequence
ISEKPWLV

SEQ ID NO: 702 - protein, 8 aa, Artificial Sequence
  Artificial peptide sequence
ISEKPWVL

SEQ ID NO: 703 - protein, 8 aa, Artificial Sequence
  Artificial peptide sequence
ISEKPWVI

SEQ ID NO: 704 - protein, 8 aa, Artificial Sequence
  Artificial peptide sequence
ISEKPWVV

SEQ ID NO: 705 - protein, 8 aa, Artificial Sequence
  Artificial peptide sequence
ISERPYIL

SEQ ID NO: 706 - protein, 8 aa, Artificial Sequence
  Artificial peptide sequence
ISERPYII

SEQ ID NO: 707 - protein, 8 aa, Artificial Sequence
  Artificial peptide sequence
ISERPYIV

SEQ ID NO: 708 - protein, 8 aa, Artificial Sequence
  Artificial peptide sequence
ISERPYLL

SEQ ID NO: 709 - protein, 8 aa, Artificial Sequence
  Artificial peptide sequence
ISERPYLI

SEQ ID NO: 710 - protein, 8 aa, Artificial Sequence
  Artificial peptide sequence
ISERPYLV

SEQ ID NO: 711 - protein, 8 aa, Artificial Sequence
  Artificial peptide sequence
ISERPYVL

SEQ ID NO: 712 - protein, 8 aa, Artificial Sequence
  Artificial peptide sequence
ISERPYVI

SEQ ID NO: 713 - protein, 8 aa, Artificial Sequence
  Artificial peptide sequence
ISERPYVV

SEQ ID NO: 714 - protein, 8 aa, Artificial Sequence
  Artificial peptide sequence
ISERPWIL

SEQ ID NO: 715 - protein, 8 aa, Artificial Sequence
  Artificial peptide sequence
ISERPWII

SEQ ID NO: 716 - protein, 8 aa, Artificial Sequence
  Artificial peptide sequence
ISERPWIV

SEQ ID NO: 717 - protein, 8 aa, Artificial Sequence
  Artificial peptide sequence
ISERPWLL

SEQ ID NO: 718 - protein, 8 aa, Artificial Sequence
  Artificial peptide sequence
ISERPWLI

SEQ ID NO: 719 - protein, 8 aa, Artificial Sequence
  Artificial peptide sequence
ISERPWLV

SEQ ID NO: 720 - protein, 8 aa, Artificial Sequence
  Artificial peptide sequence
ISERPWVL

SEQ ID NO: 721 - protein, 8 aa, Artificial Sequence
  Artificial peptide sequence
ISERPWVI

SEQ ID NO: 722 - protein, 8 aa, Artificial Sequence
  Artificial peptide sequence
ISERPWVV

SEQ ID NO: 723 - protein, 8 aa, Artificial Sequence
  Artificial peptide sequence
ITDKPYIL

SEQ ID NO: 724 - protein, 8 aa, Artificial Sequence
  Artificial peptide sequence
ITDKPYII

SEQ ID NO: 725 - protein, 8 aa, Artificial Sequence
  Artificial peptide sequence
ITDKPYIV

SEQ ID NO: 726 - protein, 8 aa, Artificial Sequence
  Artificial peptide sequence
ITDKPYLL

SEQ ID NO: 727 - protein, 8 aa, Artificial Sequence
  Artificial peptide sequence
ITDKPYLI

SEQ ID NO: 728 - protein, 8 aa, Artificial Sequence
  Artificial peptide sequence
ITDKPYLV

SEQ ID NO: 729 - protein, 8 aa, Artificial Sequence
  Artificial peptide sequence
ITDKPYVL

SEQ ID NO: 730 - protein, 8 aa, Artificial Sequence
  Artificial peptide sequence
ITDKPYVI

SEQ ID NO: 731 - protein, 8 aa, Artificial Sequence
  Artificial peptide sequence
ITDKPYVV

SEQ ID NO: 732 - protein, 8 aa, Artificial Sequence
  Artificial peptide sequence
ITDKPWIL

SEQ ID NO: 733 - protein, 8 aa, Artificial Sequence
  Artificial peptide sequence
ITDKPWII

SEQ ID NO: 734 - protein, 8 aa, Artificial Sequence
  Artificial peptide sequence
ITDKPWIV

SEQ ID NO: 735 - protein, 8 aa, Artificial Sequence
  Artificial peptide sequence
ITDKPWLL

SEQ ID NO: 736 - protein, 8 aa, Artificial Sequence
  Artificial peptide sequence
ITDKPWLI

SEQ ID NO: 737 - protein, 8 aa, Artificial Sequence
  Artificial peptide sequence
ITDKPWLV

SEQ ID NO: 738 - protein, 8 aa, Artificial Sequence
  Artificial peptide sequence
ITDKPWVL

SEQ ID NO: 739 - protein, 8 aa, Artificial Sequence
  Artificial peptide sequence
ITDKPWVI

SEQ ID NO: 740 - protein, 8 aa, Artificial Sequence
  Artificial peptide sequence
ITDKPWVV

SEQ ID NO: 741 - protein, 8 aa, Artificial Sequence
  Artificial peptide sequence
ITDRPYIL

SEQ ID NO: 742 - protein, 8 aa, Artificial Sequence
  Artificial peptide sequence
ITDRPYII

SEQ ID NO: 743 - protein, 8 aa, Artificial Sequence
  Artificial peptide sequence
ITDRPYIV

SEQ ID NO: 744 - protein, 8 aa, Artificial Sequence
  Artificial peptide sequence
ITDRPYLL

SEQ ID NO: 745 - protein, 8 aa, Artificial Sequence
  Artificial peptide sequence
ITDRPYLI

SEQ ID NO: 746 - protein, 8 aa, Artificial Sequence
  Artificial peptide sequence
ITDRPYLV

SEQ ID NO: 747 - protein, 8 aa, Artificial Sequence
  Artificial peptide sequence
ITDRPYVL

SEQ ID NO: 748 - protein, 8 aa, Artificial Sequence
  Artificial peptide sequence
ITDRPYVI

SEQ ID NO: 749 - protein, 8 aa, Artificial Sequence
  Artificial peptide sequence
ITDRPYVV

SEQ ID NO: 750 - protein, 8 aa, Artificial Sequence
  Artificial peptide sequence
ITDRPWIL

SEQ ID NO: 751 - protein, 8 aa, Artificial Sequence
  Artificial peptide sequence
ITDRPWII

SEQ ID NO: 752 - protein, 8 aa, Artificial Sequence
  Artificial peptide sequence
ITDRPWIV

SEQ ID NO: 753 - protein, 8 aa, Artificial Sequence
  Artificial peptide sequence
ITDRPWLL

SEQ ID NO: 754 - protein, 8 aa, Artificial Sequence
  Artificial peptide sequence
ITDRPWLI

SEQ ID NO: 755 - protein, 8 aa, Artificial Sequence
  Artificial peptide sequence
ITDRPWLV

SEQ ID NO: 756 - protein, 8 aa, Artificial Sequence
  Artificial peptide sequence
ITDRPWVL

SEQ ID NO: 757 - protein, 8 aa, Artificial Sequence
  Artificial peptide sequence
ITDRPWVI

SEQ ID NO: 758 - protein, 8 aa, Artificial Sequence
  Artificial peptide sequence
ITDRPWVV

SEQ ID NO: 759 - protein, 8 aa, Artificial Sequence
  Artificial peptide sequence
ITEKPYIL

SEQ ID NO: 760 - protein, 8 aa, Artificial Sequence
  Artificial peptide sequence
ITEKPYII

SEQ ID NO: 761 - protein, 8 aa, Artificial Sequence
  Artificial peptide sequence
ITEKPYIV

SEQ ID NO: 762 - protein, 8 aa, Artificial Sequence
  Artificial peptide sequence
ITEKPYLL

SEQ ID NO: 763 - protein, 8 aa, Artificial Sequence
  Artificial peptide sequence
ITEKPYLI

SEQ ID NO: 764 - protein, 8 aa, Artificial Sequence
  Artificial peptide sequence
ITEKPYLV

SEQ ID NO: 765 - protein, 8 aa, Artificial Sequence
  Artificial peptide sequence
ITEKPYVL

SEQ ID NO: 766 - protein, 8 aa, Artificial Sequence
  Artificial peptide sequence
ITEKPYVI

SEQ ID NO: 767 - protein, 8 aa, Artificial Sequence
  Artificial peptide sequence
ITEKPYVV

SEQ ID NO: 768 - protein, 8 aa, Artificial Sequence
  Artificial peptide sequence
ITEKPWIL

SEQ ID NO: 769 - protein, 8 aa, Artificial Sequence
  Artificial peptide sequence
ITEKPWII

SEQ ID NO: 770 - protein, 8 aa, Artificial Sequence
  Artificial peptide sequence
ITEKPWIV

SEQ ID NO: 771 - protein, 8 aa, Artificial Sequence
  Artificial peptide sequence
ITEKPWLL

SEQ ID NO: 772 - protein, 8 aa, Artificial Sequence
  Artificial peptide sequence
ITEKPWLI

SEQ ID NO: 773 - protein, 8 aa, Artificial Sequence
  Artificial peptide sequence
ITEKPWLV

SEQ ID NO: 774 - protein, 8 aa, Artificial Sequence
  Artificial peptide sequence
ITEKPWVL

SEQ ID NO: 775 - protein, 8 aa, Artificial Sequence
  Artificial peptide sequence
ITEKPWVI

SEQ ID NO: 776 - protein, 8 aa, Artificial Sequence
  Artificial peptide sequence
ITEKPWVV

SEQ ID NO: 777 - protein, 8 aa, Artificial Sequence
  Artificial peptide sequence
ITERPYIL

SEQ ID NO: 778 - protein, 8 aa, Artificial Sequence
  Artificial peptide sequence
ITERPYII

SEQ ID NO: 779 - protein, 8 aa, Artificial Sequence
  Artificial peptide sequence
ITERPYIV

SEQ ID NO: 780 - protein, 8 aa, Artificial Sequence
  Artificial peptide sequence
ITERPYLL

SEQ ID NO: 781 - protein, 8 aa, Artificial Sequence
  Artificial peptide sequence
ITERPYLI

SEQ ID NO: 782 - protein, 8 aa, Artificial Sequence
  Artificial peptide sequence
ITERPYLV

SEQ ID NO: 783 - protein, 8 aa, Artificial Sequence
  Artificial peptide sequence
ITERPYVL

SEQ ID NO: 784 - protein, 8 aa, Artificial Sequence
  Artificial peptide sequence
ITERPYVI

SEQ ID NO: 785 - protein, 8 aa, Artificial Sequence
  Artificial peptide sequence
ITERPYVV

SEQ ID NO: 786 - protein, 8 aa, Artificial Sequence
  Artificial peptide sequence
ITERPWIL

SEQ ID NO: 787 - protein, 8 aa, Artificial Sequence
  Artificial peptide sequence
ITERPWII

SEQ ID NO: 788 - protein, 8 aa, Artificial Sequence
  Artificial peptide sequence
ITERPWIV

SEQ ID NO: 789 - protein, 8 aa, Artificial Sequence
  Artificial peptide sequence
ITERPWLL

SEQ ID NO: 790 - protein, 8 aa, Artificial Sequence
  Artificial peptide sequence
ITERPWLI

SEQ ID NO: 791 - protein, 8 aa, Artificial Sequence
  Artificial peptide sequence
ITERPWLV

SEQ ID NO: 792 - protein, 8 aa, Artificial Sequence
  Artificial peptide sequence
ITERPWVL

SEQ ID NO: 793 - protein, 8 aa, Artificial Sequence
  Artificial peptide sequence
ITERPWVI

SEQ ID NO: 794 - protein, 8 aa, Artificial Sequence
  Artificial peptide sequence
ITERPWVV

SEQ ID NO: 795 - protein, 8 aa, Artificial Sequence
  Artificial peptide sequence
VSDKPYIL

SEQ ID NO: 796 - protein, 8 aa, Artificial Sequence
  Artificial peptide sequence
VSDKPYII

SEQ ID NO: 797 - protein, 8 aa, Artificial Sequence
  Artificial peptide sequence
VSDKPYIV

SEQ ID NO: 798 - protein, 8 aa, Artificial Sequence
  Artificial peptide sequence
VSDKPYLL

SEQ ID NO: 799 - protein, 8 aa, Artificial Sequence
  Artificial peptide sequence
VSDKPYLI

SEQ ID NO: 800 - protein, 8 aa, Artificial Sequence
  Artificial peptide sequence
VSDKPYLV

SEQ ID NO: 801 - protein, 8 aa, Artificial Sequence
  Artificial peptide sequence
VSDKPYVL

SEQ ID NO: 802 - protein, 8 aa, Artificial Sequence
  Artificial peptide sequence
VSDKPYVI

SEQ ID NO: 803 - protein, 8 aa, Artificial Sequence
  Artificial peptide sequence
VSDKPYVV

SEQ ID NO: 804 - protein, 8 aa, Artificial Sequence
  Artificial peptide sequence
VSDKPWIL

SEQ ID NO: 805 - protein, 8 aa, Artificial Sequence
  Artificial peptide sequence
VSDKPWII

SEQ ID NO: 806 - protein, 8 aa, Artificial Sequence
  Artificial peptide sequence
VSDKPWIV

SEQ ID NO: 807 - protein, 8 aa, Artificial Sequence
  Artificial peptide sequence
VSDKPWLL

SEQ ID NO: 808 - protein, 8 aa, Artificial Sequence
  Artificial peptide sequence
VSDKPWLI

SEQ ID NO: 809 - protein, 8 aa, Artificial Sequence
  Artificial peptide sequence
VSDKPWLV

SEQ ID NO: 810 - protein, 8 aa, Artificial Sequence
  Artificial peptide sequence
VSDKPWVL

SEQ ID NO: 811 - protein, 8 aa, Artificial Sequence
  Artificial peptide sequence
VSDKPWVI

SEQ ID NO: 812 - protein, 8 aa, Artificial Sequence
  Artificial peptide sequence
VSDKPWVV

SEQ ID NO: 813 - protein, 8 aa, Artificial Sequence
  Artificial peptide sequence
VSDRPYIL

SEQ ID NO: 814 - protein, 8 aa, Artificial Sequence
  Artificial peptide sequence
VSDRPYII

SEQ ID NO: 815 - protein, 8 aa, Artificial Sequence
  Artificial peptide sequence
VSDRPYIV

SEQ ID NO: 816 - protein, 8 aa, Artificial Sequence
  Artificial peptide sequence
VSDRPYLL

SEQ ID NO: 817 - protein, 8 aa, Artificial Sequence
  Artificial peptide sequence
VSDRPYLI

SEQ ID NO: 818 - protein, 8 aa, Artificial Sequence
  Artificial peptide sequence
VSDRPYLV

SEQ ID NO: 819 - protein, 8 aa, Artificial Sequence
  Artificial peptide sequence
VSDRPYVL

SEQ ID NO: 820 - protein, 8 aa, Artificial Sequence
  Artificial peptide sequence
VSDRPYVI

SEQ ID NO: 821 - protein, 8 aa, Artificial Sequence
  Artificial peptide sequence
VSDRPYVV

SEQ ID NO: 822 - protein, 8 aa, Artificial Sequence
  Artificial peptide sequence
VSDRPWIL

SEQ ID NO: 823 - protein, 8 aa, Artificial Sequence
  Artificial peptide sequence
VSDRPWII

SEQ ID NO: 824 - protein, 8 aa, Artificial Sequence
  Artificial peptide sequence
VSDRPWIV

SEQ ID NO: 825 - protein, 8 aa, Artificial Sequence
  Artificial peptide sequence
VSDRPWLL

SEQ ID NO: 826 - protein, 8 aa, Artificial Sequence
  Artificial peptide sequence
VSDRPWLI

SEQ ID NO: 827 - protein, 8 aa, Artificial Sequence
  Artificial peptide sequence
VSDRPWLV

SEQ ID NO: 828 - protein, 8 aa, Artificial Sequence
  Artificial peptide sequence
VSDRPWVL

SEQ ID NO: 829 - protein, 8 aa, Artificial Sequence
  Artificial peptide sequence
VSDRPWVI

SEQ ID NO: 830 - protein, 8 aa, Artificial Sequence
  Artificial peptide sequence
VSDRPWVV

SEQ ID NO: 831 - protein, 8 aa, Artificial Sequence
  Artificial peptide sequence
VSEKPYIL

SEQ ID NO: 832 - protein, 8 aa, Artificial Sequence
  Artificial peptide sequence
VSEKPYII

SEQ ID NO: 833 - protein, 8 aa, Artificial Sequence
  Artificial peptide sequence
VSEKPYIV

SEQ ID NO: 834 - protein, 8 aa, Artificial Sequence
  Artificial peptide sequence
VSEKPYLL

SEQ ID NO: 835 - protein, 8 aa, Artificial Sequence
  Artificial peptide sequence
VSEKPYLI

SEQ ID NO: 836 - protein, 8 aa, Artificial Sequence
  Artificial peptide sequence
VSEKPYLV

SEQ ID NO: 837 - protein, 8 aa, Artificial Sequence
  Artificial peptide sequence
VSEKPYVL

SEQ ID NO: 838 - protein, 8 aa, Artificial Sequence
  Artificial peptide sequence
VSEKPYVI

SEQ ID NO: 839 - protein, 8 aa, Artificial Sequence
  Artificial peptide sequence
VSEKPYVV

SEQ ID NO: 840 - protein, 8 aa, Artificial Sequence
  Artificial peptide sequence
VSEKPWIL

SEQ ID NO: 841 - protein, 8 aa, Artificial Sequence
  Artificial peptide sequence
VSEKPWII

SEQ ID NO: 842 - protein, 8 aa, Artificial Sequence
  Artificial peptide sequence
VSEKPWIV

SEQ ID NO: 843 - protein, 8 aa, Artificial Sequence
  Artificial peptide sequence
VSEKPWLL

SEQ ID NO: 844 - protein, 8 aa, Artificial Sequence
  Artificial peptide sequence
VSEKPWLI

SEQ ID NO: 845 - protein, 8 aa, Artificial Sequence
  Artificial peptide sequence
VSEKPWLV

SEQ ID NO: 846 - protein, 8 aa, Artificial Sequence
  Artificial peptide sequence
VSEKPWVL

SEQ ID NO: 847 - protein, 8 aa, Artificial Sequence
  Artificial peptide sequence
VSEKPWVI

SEQ ID NO: 848 - protein, 8 aa, Artificial Sequence
  Artificial peptide sequence
VSEKPWVV

SEQ ID NO: 849 - protein, 8 aa, Artificial Sequence
  Artificial peptide sequence
VSERPYIL

SEQ ID NO: 850 - protein, 8 aa, Artificial Sequence
  Artificial peptide sequence
VSERPYII

SEQ ID NO: 851 - protein, 8 aa, Artificial Sequence
  Artificial peptide sequence
VSERPYIV

SEQ ID NO: 852 - protein, 8 aa, Artificial Sequence
  Artificial peptide sequence
VSERPYLL

SEQ ID NO: 853 - protein, 8 aa, Artificial Sequence
  Artificial peptide sequence
VSERPYLI

SEQ ID NO: 854 - protein, 8 aa, Artificial Sequence
  Artificial peptide sequence
VSERPYLV

SEQ ID NO: 855 - protein, 8 aa, Artificial Sequence
  Artificial peptide sequence
VSERPYVL

SEQ ID NO: 856 - protein, 8 aa, Artificial Sequence
  Artificial peptide sequence
VSERPYVI

SEQ ID NO: 857 - protein, 8 aa, Artificial Sequence
  Artificial peptide sequence
VSERPYVV

SEQ ID NO: 858 - protein, 8 aa, Artificial Sequence
  Artificial peptide sequence
VSERPWIL

SEQ ID NO: 859 - protein, 8 aa, Artificial Sequence
  Artificial peptide sequence
VSERPWII

SEQ ID NO: 860 - protein, 8 aa, Artificial Sequence
  Artificial peptide sequence
VSERPWIV

SEQ ID NO: 861 - protein, 8 aa, Artificial Sequence
  Artificial peptide sequence
VSERPWLL

SEQ ID NO: 862 - protein, 8 aa, Artificial Sequence
  Artificial peptide sequence
VSERPWLI

SEQ ID NO: 863 - protein, 8 aa, Artificial Sequence
  Artificial peptide sequence
VSERPWLV

SEQ ID NO: 864 - protein, 8 aa, Artificial Sequence
  Artificial peptide sequence
VSERPWVL

SEQ ID NO: 865 - protein, 8 aa, Artificial Sequence
  Artificial peptide sequence
VSERPWVI

SEQ ID NO: 866 - protein, 8 aa, Artificial Sequence
  Artificial peptide sequence
VSERPWVV

SEQ ID NO: 867 - protein, 8 aa, Artificial Sequence
  Artificial peptide sequence
VTDKPYIL

SEQ ID NO: 868 - protein, 8 aa, Artificial Sequence
  Artificial peptide sequence
VTDKPYII

SEQ ID NO: 869 - protein, 8 aa, Artificial Sequence
  Artificial peptide sequence
VTDKPYIV

SEQ ID NO: 870 - protein, 8 aa, Artificial Sequence
  Artificial peptide sequence
VTDKPYLL

SEQ ID NO: 871 - protein, 8 aa, Artificial Sequence
  Artificial peptide sequence
VTDKPYLI

SEQ ID NO: 872 - protein, 8 aa, Artificial Sequence
  Artificial peptide sequence
VTDKPYLV

SEQ ID NO: 873 - protein, 8 aa, Artificial Sequence
  Artificial peptide sequence
VTDKPYVL

SEQ ID NO: 874 - protein, 8 aa, Artificial Sequence
  Artificial peptide sequence
VTDKPYVI

SEQ ID NO: 875 - protein, 8 aa, Artificial Sequence
  Artificial peptide sequence
VTDKPYVV

SEQ ID NO: 876 - protein, 8 aa, Artificial Sequence
  Artificial peptide sequence
VTDKPWIL

SEQ ID NO: 877 - protein, 8 aa, Artificial Sequence
  Artificial peptide sequence
VTDKPWII

SEQ ID NO: 878 - protein, 8 aa, Artificial Sequence
  Artificial peptide sequence
VTDKPWIV

SEQ ID NO: 879 - protein, 8 aa, Artificial Sequence
  Artificial peptide sequence
VTDKPWLL

SEQ ID NO: 880 - protein, 8 aa, Artificial Sequence
  Artificial peptide sequence
VTDKPWLI

SEQ ID NO: 881 - protein, 8 aa, Artificial Sequence
  Artificial peptide sequence
VTDKPWLV

SEQ ID NO: 882 - protein, 8 aa, Artificial Sequence
  Artificial peptide sequence
VTDKPWVL

SEQ ID NO: 883 - protein, 8 aa, Artificial Sequence
  Artificial peptide sequence
VTDKPWVI

SEQ ID NO: 884 - protein, 8 aa, Artificial Sequence
  Artificial peptide sequence
VTDKPWVV

SEQ ID NO: 885 - protein, 8 aa, Artificial Sequence
  Artificial peptide sequence
VTDRPYIL

SEQ ID NO: 886 - protein, 8 aa, Artificial Sequence
  Artificial peptide sequence
VTDRPYII

SEQ ID NO: 887 - protein, 8 aa, Artificial Sequence
  Artificial peptide sequence
VTDRPYIV

SEQ ID NO: 888 - protein, 8 aa, Artificial Sequence
  Artificial peptide sequence
VTDRPYLL

SEQ ID NO: 889 - protein, 8 aa, Artificial Sequence
  Artificial peptide sequence
VTDRPYLI

SEQ ID NO: 890 - protein, 8 aa, Artificial Sequence
  Artificial peptide sequence
VTDRPYLV

SEQ ID NO: 891 - protein, 8 aa, Artificial Sequence
  Artificial peptide sequence
VTDRPYVL

SEQ ID NO: 892 - protein, 8 aa, Artificial Sequence
  Artificial peptide sequence
VTDRPYVI

SEQ ID NO: 893 - protein, 8 aa, Artificial Sequence
  Artificial peptide sequence
VTDRPYVV

SEQ ID NO: 894 - protein, 8 aa, Artificial Sequence
  Artificial peptide sequence
VTDRPWIL

SEQ ID NO: 895 - protein, 8 aa, Artificial Sequence
  Artificial peptide sequence
VTDRPWII

SEQ ID NO: 896 - protein, 8 aa, Artificial Sequence
  Artificial peptide sequence
VTDRPWIV

SEQ ID NO: 897 - protein, 8 aa, Artificial Sequence
  Artificial peptide sequence
VTDRPWLL

SEQ ID NO: 898 - protein, 8 aa, Artificial Sequence
  Artificial peptide sequence
VTDRPWLI

SEQ ID NO: 899 - protein, 8 aa, Artificial Sequence
  Artificial peptide sequence
VTDRPWLV

SEQ ID NO: 900 - protein, 8 aa, Artificial Sequence
  Artificial peptide sequence
VTDRPWVL

SEQ ID NO: 901 - protein, 8 aa, Artificial Sequence
  Artificial peptide sequence
VTDRPWVI

SEQ ID NO: 902 - protein, 8 aa, Artificial Sequence
  Artificial peptide sequence
VTDRPWVV

SEQ ID NO: 903 - protein, 8 aa, Artificial Sequence
  Artificial peptide sequence
VTEKPYIL

SEQ ID NO: 904 - protein, 8 aa, Artificial Sequence
  Artificial peptide sequence
VTEKPYII

SEQ ID NO: 905 - protein, 8 aa, Artificial Sequence
  Artificial peptide sequence
VTEKPYIV

SEQ ID NO: 906 - protein, 8 aa, Artificial Sequence
  Artificial peptide sequence
VTEKPYLL

SEQ ID NO: 907 - protein, 8 aa, Artificial Sequence
  Artificial peptide sequence
VTEKPYLI

SEQ ID NO: 908 - protein, 8 aa, Artificial Sequence
  Artificial peptide sequence
VTEKPYLV

SEQ ID NO: 909 - protein, 8 aa, Artificial Sequence
  Artificial peptide sequence
VTEKPYVL

SEQ ID NO: 910 - protein, 8 aa, Artificial Sequence
  Artificial peptide sequence
VTEKPYVI

SEQ ID NO: 911 - protein, 8 aa, Artificial Sequence
  Artificial peptide sequence
VTEKPYVV

SEQ ID NO: 912 - protein, 8 aa, Artificial Sequence
  Artificial peptide sequence
VTEKPWIL

SEQ ID NO: 913 - protein, 8 aa, Artificial Sequence
  Artificial peptide sequence
VTEKPWII

SEQ ID NO: 914 - protein, 8 aa, Artificial Sequence
  Artificial peptide sequence
VTEKPWIV

SEQ ID NO: 915 - protein, 8 aa, Artificial Sequence
  Artificial peptide sequence
VTEKPWLL

SEQ ID NO: 916 - protein, 8 aa, Artificial Sequence
  Artificial peptide sequence
VTEKPWLI

SEQ ID NO: 917 - protein, 8 aa, Artificial Sequence
  Artificial peptide sequence
VTEKPWLV

SEQ ID NO: 918 - protein, 8 aa, Artificial Sequence
  Artificial peptide sequence
VTEKPWVL

SEQ ID NO: 919 - protein, 8 aa, Artificial Sequence
  Artificial peptide sequence
VTEKPWVI

SEQ ID NO: 920 - protein, 8 aa, Artificial Sequence
  Artificial peptide sequence
VTEKPWVV

SEQ ID NO: 921 - protein, 8 aa, Artificial Sequence
  Artificial peptide sequence
VTERPYIL

SEQ ID NO: 922 - protein, 8 aa, Artificial Sequence
  Artificial peptide sequence
VTERPYII

SEQ ID NO: 923 - protein, 8 aa, Artificial Sequence
  Artificial peptide sequence
VTERPYIV

SEQ ID NO: 924 - protein, 8 aa, Artificial Sequence
  Artificial peptide sequence
VTERPYLL

SEQ ID NO: 925 - protein, 8 aa, Artificial Sequence
  Artificial peptide sequence
VTERPYLI

SEQ ID NO: 926 - protein, 8 aa, Artificial Sequence
  Artificial peptide sequence
VTERPYLV

SEQ ID NO: 927 - protein, 8 aa, Artificial Sequence
  Artificial peptide sequence
VTERPYVL

SEQ ID NO: 928 - protein, 8 aa, Artificial Sequence
  Artificial peptide sequence
VTERPYVI

SEQ ID NO: 929 - protein, 8 aa, Artificial Sequence
  Artificial peptide sequence
VTERPYVV

SEQ ID NO: 930 - protein, 8 aa, Artificial Sequence
  Artificial peptide sequence
VTERPWIL

SEQ ID NO: 931 - protein, 8 aa, Artificial Sequence
  Artificial peptide sequence
VTERPWII

SEQ ID NO: 932 - protein, 8 aa, Artificial Sequence
  Artificial peptide sequence
VTERPWIV

SEQ ID NO: 933 - protein, 8 aa, Artificial Sequence
  Artificial peptide sequence
VTERPWLL

SEQ ID NO: 934 - protein, 8 aa, Artificial Sequence
  Artificial peptide sequence
VTERPWLI

SEQ ID NO: 935 - protein, 8 aa, Artificial Sequence
  Artificial peptide sequence
VTERPWLV

SEQ ID NO: 936 - protein, 8 aa, Artificial Sequence
  Artificial peptide sequence
VTERPWVL

SEQ ID NO: 937 - protein, 8 aa, Artificial Sequence
  Artificial peptide sequence
VTERPWVI

SEQ ID NO: 938 - protein, 8 aa, Artificial Sequence
  Artificial peptide sequence
VTERPWVV

SEQ ID NO: 939 - protein, 8 aa, Artificial Sequence
  Artificial peptide sequence
YSDKPYIL

SEQ ID NO: 940 - protein, 8 aa, Artificial Sequence
  Artificial peptide sequence
WSDKPYIL

SEQ ID NO: 941 - protein, 8 aa, Artificial Sequence
  Artificial peptide sequence
TSDKPYIL

SEQ ID NO: 942 - protein, 8 aa, Artificial Sequence
  Artificial peptide sequence
SSDKPYIL

SEQ ID NO: 943 - protein, 8 aa, Artificial Sequence
  Artificial peptide sequence
RSDKPYIL

SEQ ID NO: 944 - protein, 8 aa, Artificial Sequence
  Artificial peptide sequence
QSDKPYIL

SEQ ID NO: 945 - protein, 8 aa, Artificial Sequence
  Artificial peptide sequence
PSDKPYIL

SEQ ID NO: 946 - protein, 8 aa, Artificial Sequence
  Artificial peptide sequence
NSDKPYIL

SEQ ID NO: 947 - protein, 8 aa, Artificial Sequence
  Artificial peptide sequence
MSDKPYIL

SEQ ID NO: 948 - protein, 8 aa, Artificial Sequence
  Artificial peptide sequence
KSDKPYIL

SEQ ID NO: 949 - protein, 8 aa, Artificial Sequence
  Artificial peptide sequence
HSDKPYIL

SEQ ID NO: 950 - protein, 8 aa, Artificial Sequence
  Artificial peptide sequence
GSDKPYIL

SEQ ID NO: 951 - protein, 8 aa, Artificial Sequence
  Artificial peptide sequence
FSDKPYIL

SEQ ID NO: 952 - protein, 8 aa, Artificial Sequence
  Artificial peptide sequence
ESDKPYIL

SEQ ID NO: 953 - protein, 8 aa, Artificial Sequence
  Artificial peptide sequence
DSDKPYIL

SEQ ID NO: 954 - protein, 8 aa, Artificial Sequence
  Artificial peptide sequence
CSDKPYIL

SEQ ID NO: 955 - protein, 7 aa, Artificial Sequence
  Artificial peptide sequence
YDKPYIL

SEQ ID NO: 956 - protein, 7 aa, Artificial Sequence
  Artificial peptide sequence
WDKPYIL

SEQ ID NO: 957 - protein, 7 aa, Artificial Sequence
  Artificial peptide sequence
VDKPYIL

SEQ ID NO: 958 - protein, 7 aa, Artificial Sequence
  Artificial peptide sequence
RDKPYIL

SEQ ID NO: 959 - protein, 7 aa, Artificial Sequence
  Artificial peptide sequence
QDKPYIL

SEQ ID NO: 960 - protein, 7 aa, Artificial Sequence
  Artificial peptide sequence
PDKPYIL

SEQ ID NO: 961 - protein, 7 aa, Artificial Sequence
  Artificial peptide sequence
NDKPYIL

SEQ ID NO: 962 - protein, 7 aa, Artificial Sequence
  Artificial peptide sequence
MDKPYIL

SEQ ID NO: 963 - protein, 7 aa, Artificial Sequence
  Artificial peptide sequence
LDKPYIL

SEQ ID NO: 964 - protein, 7 aa, Artificial Sequence
  Artificial peptide sequence
KDKPYIL

SEQ ID NO: 965 - protein, 7 aa, Artificial Sequence
  Artificial peptide sequence
IDKPYIL

SEQ ID NO: 966 - protein, 7 aa, Artificial Sequence
  Artificial peptide sequence
HDKPYIL

SEQ ID NO: 967 - protein, 7 aa, Artificial Sequence
  Artificial peptide sequence
GDKPYIL

SEQ ID NO: 968 - protein, 7 aa, Artificial Sequence
  Artificial peptide sequence
FDKPYIL

SEQ ID NO: 969 - protein, 7 aa, Artificial Sequence
  Artificial peptide sequence
EDKPYIL

SEQ ID NO: 970 - protein, 7 aa, Artificial Sequence
  Artificial peptide sequence
DDKPYIL

SEQ ID NO: 971 - protein, 7 aa, Artificial Sequence
  Artificial peptide sequence
CDKPYIL

SEQ ID NO: 972 - protein, 7 aa, Artificial Sequence
  Artificial peptide sequence
ADKPYIL

SEQ ID NO: 973 - protein, 6 aa, Artificial Sequence
  Artificial peptide sequence
YKPYIL

SEQ ID NO: 974 - protein, 6 aa, Artificial Sequence
  Artificial peptide sequence
WKPYIL

SEQ ID NO: 975 - protein, 6 aa, Artificial Sequence
  Artificial peptide sequence
VKPYIL

SEQ ID NO: 976 - protein, 6 aa, Artificial Sequence
  Artificial peptide sequence
TKPYIL

SEQ ID NO: 977 - protein, 6 aa, Artificial Sequence
  Artificial peptide sequence
SKPYIL

SEQ ID NO: 978 - protein, 6 aa, Artificial Sequence
  Artificial peptide sequence
QKPYIL

SEQ ID NO: 979 - protein, 6 aa, Artificial Sequence
  Artificial peptide sequence
PKPYIL

SEQ ID NO: 980 - protein, 6 aa, Artificial Sequence
  Artificial peptide sequence
NKPYIL

SEQ ID NO: 981 - protein, 6 aa, Artificial Sequence
  Artificial peptide sequence
MKPYIL

SEQ ID NO: 982 - protein, 6 aa, Artificial Sequence
  Artificial peptide sequence
LKPYIL

SEQ ID NO: 983 - protein, 6 aa, Artificial Sequence
  Artificial peptide sequence
IKPYIL

SEQ ID NO: 984 - protein, 6 aa, Artificial Sequence
  Artificial peptide sequence
HKPYIL

SEQ ID NO: 985 - protein, 6 aa, Artificial Sequence
  Artificial peptide sequence
FKPYIL

SEQ ID NO: 986 - protein, 6 aa, Artificial Sequence
  Artificial peptide sequence
CKPYIL

SEQ ID NO: 987 - protein, 6 aa, Artificial Sequence
  Artificial peptide sequence
AKPYIL

SEQ ID NO: 988 - protein, 5 aa, Artificial Sequence
  Artificial peptide sequence
YPYIL

SEQ ID NO: 989 - protein, 5 aa, Artificial Sequence
  Artificial peptide sequence
WPYIL

SEQ ID NO: 990 - protein, 5 aa, Artificial Sequence
  Artificial peptide sequence
VPYIL

SEQ ID NO: 991 - protein, 5 aa, Artificial Sequence
  Artificial peptide sequence
TPYIL

SEQ ID NO: 992 - protein, 5 aa, Artificial Sequence
  Artificial peptide sequence
SPYIL

SEQ ID NO: 993 - protein, 5 aa, Artificial Sequence
  Artificial peptide sequence
QPYIL

SEQ ID NO: 994 - protein, 5 aa, Artificial Sequence
  Artificial peptide sequence
PPYIL

SEQ ID NO: 995 - protein, 5 aa, Artificial Sequence
  Artificial peptide sequence
NPYIL

SEQ ID NO: 996 - protein, 5 aa, Artificial Sequence
  Artificial peptide sequence
MPYIL

SEQ ID NO: 997 - protein, 5 aa, Artificial Sequence
  Artificial peptide sequence
LPYIL

SEQ ID NO: 998 - protein, 5 aa, Artificial Sequence
  Artificial peptide sequence
IPYIL

SEQ ID NO: 999 - protein, 5 aa, Artificial Sequence
  Artificial peptide sequence
HPYIL

SEQ ID NO: 1000 - protein, 5 aa, Artificial Sequence
  Artificial peptide sequence
GPYIL

SEQ ID NO: 1001 - protein, 5 aa, Artificial Sequence
  Artificial peptide sequence
FPYIL

SEQ ID NO: 1002 - protein, 5 aa, Artificial Sequence
  Artificial peptide sequence
EPYIL

SEQ ID NO: 1003 - protein, 5 aa, Artificial Sequence
  Artificial peptide sequence
DPYIL

SEQ ID NO: 1004 - protein, 5 aa, Artificial Sequence
  Artificial peptide sequence
CPYIL

SEQ ID NO: 1005 - protein, 5 aa, Artificial Sequence
  Artificial peptide sequence
APYIL